European Patent Specification EP 3 728 632 B1, published July 12, 2023. Title: MOLECULE D'ADN DOUBLE-BRIN POUR LA DETECTION ET LA CARACTERISATION DES INTERACTIONS MOLECULAIRES. Applicant: PARIS SCIENCES ET LETTRES - QUARTIER LATIN CENTRE NATIONAL DE LA RECHERCHE SCIENTIFIQUE ECOLE NORMALE SUPERIEURE UNIVERSITE PARIS DIDEROT PARIS 7 INSTITUT NATIONAL DE LA SANTE ET DE LA RECHERCHE MEDICALE. The sequence listing filed with the application follows.

SEQUENCE LISTING (50 sequences)

SEQ ID NO: 1 - DNA, 2285 bp, Artificial
  Produit d'amplification pour utilisation en tant qu'éxtrémités pour l'attachement de la molécule aux supports
gcgtattagcgacccatcgtctttctgatttaataatagatgattcagttaaatatgaaggtaatttcttttgtgcaagtctgactaacttttttataccaatgtttaacatactttcatttgtaataaactcaatgtcattttcttcaatgtaagatgaaataagagtagcctttgcctcgctatacatttctaaatcgccttgtttttctatcgtattgcgagaatttttagcccaagccattaatggatcatttttccatttttcaataacattattgttataccaaatgtcatatcctataatctggtttttgtttttttgaataataaatgttactgttcttgcggtttggaggaattgattcaaattcaagcgaaataattcagggtcaaaatatgtatcaatgcagcatttgagcaagtgcgataaatctttaagtcttctttcccatggttttttagtcataaaactctccattttgataggttgcatgctagatgctgatatattttagaggtgataaaattaactgcttaactgtcaatgtaatacaagttgtttgatctttgcaatgattcttatcagaaaccatatagtaaattagttacacaggaaatttttaatattattattatcattcattatgtattaaaattagagttgtggcttggctctgctaacacgttgctcataggagatatggtagagccgcagacacgtcgtatgcaggaacgtgctgcggctggctggtgaacttccgatagtgcgggtgttgaatgatttccagttgctaccgattttacatattttttgcatgagagaatttgtaccacctcccaccgaccatctatgactgtacgccactgtccctaggactgctatgtgccggagcggacattacaaacgtccttctcggtgcatgccactgttgccaatgacctgcctaggaattggttagcaagttactaccggattttgtaaaaacagccctcctcatataaaaagtattcgttcacttccgataagcgtcgtaattttctatctttcatcatattctagatccctctgaaaaaatcttccgagtttgctaggcactgatacataactcttttccaataattggggaagtcattcaaatctataataggtttcagatttgcttcaataaattctgactgtagctgctgaaacgttgcggttgaactatatttccttataacttttacgaaagagtttctttgagtaatcacttcactcaagtgcttccctgcctccaaacgatacctgttagcaatatttaatagcttgaaatgatgaagagctctgtgtttgtcttcctgcctccagttcgccgggcattcaacataaaaactgatagcacccggagttccggaaacgaaatttgcatatacccattgctcacgaaaaaaaatgtccttgtcgatatagggatgaatcgcttggtgtacctcatctactgcgaaaacttgacctttctctcccatattgcagtcgcggcacgatggaactaaattaataggcatcaccgaaaattcaggataatgtgcaataggaagaaaatgatctatattttttgtctgtcctatatcaccacaaaatggacatttttcacctgatgaaacaagcatgtcatcgtaatatgttctagcgggtttgtttttatctcggagattattttcataaagcttttctaatttaacctttgtcaggttaccaactactaaggttgtaggctcaagagggtgtgtcctgtcgtaggtaaataactgacctgtcgagcttaatattctatattgttgttctttctgcaaaaaagtggggaagtgagtaatgaaattatttctaacatttatctgcatcataccttccgagcatttattaagcatttcgctataagttctcgctggaagaggtagttttttcattgtactttaccttcatctctgttcattatcatcgcttttaaaacggttcgaccttctaatcctatctgaccattataattttttagaatggtttcataagaaagctctgaatcaacggactgcgataataagtggtggtatccagaatttgtcacttcaagtaaaaacacctcacgagttaaaacacctaagttctcaccgaatgtctcaatatccggacggataatatttattgcttctcttgaccgtaggactttccacatgcaggattttggaacctcttgcagtactactggggaatgagttgcaattattgctacaccattgcgtgcatc

SEQ ID NO: 2 - DNA, 27 bp, Artificial
  Oligo - forward pour amplication de l'extrémité pour l'attachement à un support
gcgtattagcgacccatcgtctttctg

SEQ ID NO: 3 - DNA, 29 bp, Artificial
  Oligo - reverse pour amplication de l'extrémité pour l'attachement à un support
gatgcacgcaatggtgtagcaataattgc

SEQ ID NO: 4 - DNA, 10 bp, Artificial
  Oligo-TC1
tatatgaggc

SEQ ID NO: 5 - DNA, 10 bp, Artificial
  Oligo-TC2
ttgtaagagc

SEQ ID NO: 6 - protein, 104 aa, Artificial
  Proteine FRB comprenant un résidu de clivage GPLGS en N-ter
GPLGSFILWHEMWHEGLEEASRLYFGERNVKGMFEVLEPLHAMMERGPQTLKETSFNQAYGRDLMEAQEWCRKYMKSGNVKDLTQAWDLYYHVFRRISKQLPQL

SEQ ID NO: 7 - protein, 113 aa, Artificial
  Proteine FKBP12 comprenant un résidu de clivage GPLGS en N-ter
GPLGSFGVQVETISPGDGRTFPKRGQTCVVHYTGMLEDGKKFDSSRDRNKPFKFMLGKQEVIRGWEEGVAQMSVGQRAKLTISPDYAYGATGHPGIIPPHATLVFDVELLKLE

SEQ ID NO: 8 - DNA, 5287 bp, Artificial
  Charomid 9-5 DSbfI plasmid
gaattcgagctcggtacccggggatcctctagagtcaacagcagaaacatacaagctgtcagctttgcacaagggcccaacaccctgctcatcaagaagcactgtggttgctgtgttagtaatgtgcaaaacaggaggcacattttccccacctgtgtaggttccaaaatatctagtgttttcatttttacttggatcaggaacccagcactccactggataagcattatccttatccaaaacagccttgtggtcagtgttcatctgctgactgtcgacctgcatgcaggcatgcaagctttaatgcggtagtttatcacagttaaattgctaacgcagtcaggcaccgtgtatgaaatctaacaatgcgctcatcgtcatcctcggcaccgtcaccctggatgctgtaggcataggcttggttatgccggtactgccgggcctcttgcgggatatcgtccattccgacagcatcgccagtcactatggcgtgctgctagcgctatatgcgttgatgcaatttctatgcgcacccgttctcggagcactgtccgaccgctttggccgccgcccagtcctgctcgcttcgctacttggagccactatcgactacgcgatcatggcgaccacacccgtcctgtggatctgcctcgttggcctgccgcagttcttcaacctcccggcgcagcttttcgttctcaatttcagcatccctttcggcataccattttatgacggcggcagagtcataaagcacctcattacccttgccaccgcctcgcagaacgggcattccctgttcctgccagttctgaatggtacggatactcgcaccgaaaatgtcagccagctgctttttgttgacttccattgttcattccacggacaaaaacagagaaaggaaacgacagaggccaaaaagctcgctttcagcacctgtcgtttcctttcttttcagagggtattttaaataaaaacattaagttatgacgaagaagaacggaaacgccttaaaccggaaaattttcataaatagcgaaaacccgcgaggtcgccgccccgtaacaaggcggatcgccggaaaggacccgcaaatgataataattatcaattgcatactatcgacggcactgctgccagataacaccaccggggaaacattccatcatgatggccgtgcggacataggaagccagttcatccatcgctttcttgtctgctgccatttgctttgtgacatccagcgccgcacattcagcagcgtttttcagcgcgttttcgatcaacgtttcaatgttggtatcaacaccaggtttaactttgaacttatcggcactgacggttaccttgttctgcgctggctcatcacgctggataccaaggctgatgttgtagatattggtcaccggctgaggtgtttcgattgccgctgcgtggatagcaccatttgcgatagcggcgtccttgatgaatgacactccattgcgaataagttcgaaggagacggtgtcacgaatgcgctggtccagctcgtcgattgccttttgtgcagcagaggtatcaatctcaacgccaagcgtcatcgaagcgcaatattgctgctcaccaaaacgcgtattgaccaggtgttcaacggcaaatttctgcccttctgatgtcagaaaggtaaagtgattttctttctggtattcagttgctgtgtgtctggtttcagcaaaaccaagctcgcgcaattcggctgtgccagatttagaaggcagatcaccagacagcaacgcgccacggaaaaacagcgcatacagaacatccgtcgccgcgccggacaacgtgataattttatgacccatgatttatttccttttagacgtgagcctgtcgcacagcaaagccgccgaaagttaacggtttgcccaggctcacaactgaaagactttctacggtgtgcgcgtgcgatgcgcgtagaagactgatttatcaacctgtctttatatcaggattcattacctgactatttgtgggtaaagttcgtagtgcgctgatcgtgcaaaatgattttagttgggaacagttcgcaactctgtcccataaaaatcagcatattcccatctatcccatatccagcgcattgaccatcgggatactgaagggagattccatcatctcttagaaagatcaccatctcttttgtttcaatttgcatatagctacctggaggatttatgaatacaaggattttcatggactattaccatgagattgattttccatctttattcgcgagagcagtggaaagcgatgacgatgtgggtactacattgcgcattcacctactttgtgagcgcatggtcgaagcatggatatgcgcatgctgtgactgccaagatcctctacgccggacgcatcgtggccggcatcaccggcgccacaggtgcggttgctggcgcctatatcgccgacatcaccgatggggaagatcgggctcgccacttcgggctcatgagcgcttgtttcggcgtgggtatggtggcaggccccgtggccgggggactgttgggcgccatctccttgcatgcaccattccttgcggcggcggtgctcaacggcctcaacctactactgggctgcttcctaatgcaggagtcgcataagggagagcgtcgaccgatgcccttgagagccttcaacccagtcagctccttccggtgggcgcggggcatgactatcgtcgccgcacttatgactgtcttctttatcatgcaactcgtaggacaggtgccggcagcgctctgggtcattttcggcgaggaccgctttcgctggagcgcgacgatgatcggcctgtcgcttgcggtattcggaatcttgcacgccctcgctcaagccttcgtcactggtcccgccaccaaacgtttcggcgagaagcaggccattatcgccggcatggcggccgacgcgctgggctacgtcttgctggcgttcgcgacgcgaggctggatggccttccccattatgattcttctcgcttccggcggcatcgggatgcccgcgttgcaggccatgctgtccaggcaggtagatgacgaccatcagggacagcttcaaggatcgctcgcggctcttaccagcctaacttcgatcattggaccgctgatcgtcacggcgatttatgccgcctcggcgagcacatggaacgggttggcatggattgtaggcgccgccctataccttgtctgcctccccgcgttgcgtcgcggtgcatggagccgggccacctcgacctgaatggaagccggcggcacctcgctaacggattcaccactccaagaattggagccaatcaattcttgcggagaactgtgaatgcgcaaaccaacccttggcagaacatatccatcgcgtccgccatctccagcagccgcacgcggcgcatctcgggccgcgttgctggcgtttttccataggctccgcccccctgacgagcatcacaaaaatcgacgctcaagtcagaggtggcgaaacccgacaggactataaagataccaggcgtttccccctggaagctccctcgtgcgctctcctgttccgaccctgccgcttaccggatacctgtccgcctttctcccttcgggaagcgtggcgctttctcatagctcacgctgtaggtatctcagttcggtgtaggtcgttcgctccaagctgggctgtgtgcacgaaccccccgttcagcccgaccgctgcgccttatccggtaactatcgtcttgagtccaacccggtaagacacgacttatcgccactggcagcagccactggtaacaggattagcagagcgaggtatgtaggcggtgctacagagttcttgaagtggtggcctaactacggctacactagaaggacagtatttggtatctgcgctctgctgaagccagttaccttcggaaaaagagttggtagctcttgatccggcaaacaaaccaccgctggtagcggtggtttttttgtttgcaagcagcagattacgcgcagaaaaaaaggatctcaagaagatcctttgatcttttctacggggtctgacgctcagtggaacgaaaactcacgttaagggattttggtcatgagattatcaaaaaggatcttcacctagatccttttaaattaaaaatgaagttttaaatcaatctaaagtatatatgagtaaacttggtctgacagttaccaatgcttaatcagtgaggcacctatctcagcgatctgtctatttcgttcatcccatagttgcctgcaactccccgtcgtgtagataactacgatacgggagggcttaccatctggccccagtgctgcaatgataccgcgaagacccacgctcaccggctccagatttatcagcaataaaccagccagccggaagggccgagcgcagaagtggtcctgcaactttatccgcctccatccagtctattaattgttgccgggaagctagagtaagtagttcgccagttaatagtttgcgcaacgttgttgccattgctgcaggcatcgtggtgtcacgctcgtcgtttggtatggcttcattcagctccggttcccaacgatcaaggcgagttacatgatcccccatgttgtgcaaaaaagcggttagctccttcggtcctccgatcgttgtcagaagtaagttggccgcagtgttatcactcatggttatggcagcactgcataattctcttactgtcatgccatccgtaagatgcttttctgtgactggtgagtactcaaccaagtcattctgagaatagtgtatgcggcgaccgagttgctcttgcccggcgtcaacacgggataataccgcgccacatagcagaactttaaaagtgctcatcattggaaaacgttcttcggggcgaaaactctcaaggatcttaccgctgttgagatccagttcgatgtaacccactcgtgcacccaactgatcttcagcatcttttactttcaccagcgtttctgggtgagcaaaaacaggaaggcaaaatgccgcaaaaaagggaataagggcgacacggaaatgttgaatactcatactcttcctttttcaatattattgaagcatttatcagggttattgtctcatgagcggatacatatttgaatgtatttagaaaaataaacaaataggggttccgcgcacatttccccgaaaagtgccacctgacgtctaagaaaccattattatcatgacattaacctataaaaataggcgtatcacgaggccctttcgtcttcaagaattc

SEQ ID NO: 9 - DNA, 3040 bp, Artificial
  Molecule (A), Exemples 8 et 9
gagagacccgggcacgacttatcgccactggcagcagccactggtaacaggattagcagagcgaggtatgtaggcggtgctacagagttcttgaagtggtggcctaactacggctacactagaaggacagtatttggtatctgcgctctgctgaagccagttaccttcggaaaaagagttggtagctcttgatccggcaaacaaaccaccgctggtagcggtggtttttttgtttgcaagcagcagattacgcgcagaaaaaaaggatctcaagaagatcctttgatcttttctacggggtctgacgctcagtggaacgaaaactcacgttaagggattttggtcatgagattatcaaaaaggatcttcacctagatccttttaaattaaaaatgaagttttaaatcaatctaaagtatatatgagtaaacttggtctgacagttaccaatgcttaatcagtgaggcacctatctcagcgatctgtctatttcgttcatcccatagttgcctgcaactccccgtcgtgtagataactacgatacgggagggcttaccatctggccccagtgctgcaatgataccgcgaagacccacgctcaccggctccagatttatcagcaataaaccagccagccggaagggccgagcgcagaagtggtcctgcaactttatccgcctccatccagtctattaattgttgccgggaagctagagtaagtagttcgccagttaatagtttgcgcaacgttgttgccattgctgcaggcatcgtggtgtcacgctcgtcgtttggtatggcttcattcagctccggttcccaacgatcaaggcgagttacatgatcccccatgttgtgcaaaaaagcggttagctccttcggtcctccgatcgttgtcagaagtaagttggccgcagtgttatcactcatggttatggcagcactgcataattctcttactgtcatgccatccgtaagatgcttttctgtgactggtgagtactcaaccaagtcattctgagaatagtgtatgcggcgaccgagttgctcttgcccggcgtcaacacgggataataccgcgccacatagcagaactttaaaagtgctcatcattggaaaacgttcttcggggcgaaaactctcaaggatcttaccgctgttgagatccagttcgatgtaacccactcgtgcacccaactgatcttcagcatcttttactttcaccagcgtttctgggtgagcaaaaacaggaaggcaaaatgccgcaaaaaagggaataagggcgacacggaaatgttgaatactcatactcttcctttttcaatattattgaagcatttatcagggttattgtctcatgagcggatacatatttgaatgtatttagaaaaataaacaaataggggttccgcgcacatttccccgaaaagtgccacctgacgtctaagaaaccattattatcatgacattaacctataaaaataggcgtatcacgaggccctttcgtcttcaagaattcgaattcgagctcggtacccggggatcctctagagtcaacagcagaaacatacaagctgtcagctttgcacaagggcccaacaccctgctcatcaagaagcactgtggttgctgtgttagtaatgtgcaaaacaggaggcacattttccccacctgtgtaggttccaaaatatctagtgttttcatttttacttggatcaggaacccagcactccactggataagcattatccttatccaaaacagccttgtggtcagtgttcatctgctgactgtcgacctgcatgcaggcatgcaagctttaatgcggtagtttatcacagttaaattgctaacgcagtcaggcaccgtgtatgaaatctaacaatgcgctcatcgtcatcctcggcaccgtcaccctggatgctgtaggcataggcttggttatgccggtactgccgggcctcttgcgggatatcgtccattccgacagcatcgccagtcactatggcgtgctgctagcgctatatgcgttgatgcaatttctatgcgcacccgttctcggagcactgtccgaccgctttggccgccgcccagtcctgctcgcttcgctacttggagccactatcgactacgcgatcatggcgaccacacccgtcctgtggatctgcctcgttggcctgccgcagttcttcaacctcccggcgcagcttttcgttctcaatttcagcatccctttcggcataccattttatgacggcggcagagtcataaagcacctcattacccttgccaccgcctcgcagaacgggcattccctgttcctgccagttctgaatggtacggatactcgcaccgaaaatgtcagccagctgctttttgttgacttccattgttcattccacggacaaaaacagagaaaggaaacgacagaggccaaaaagctcgctttcagcacctgtcgtttcctttcttttcagagggtattttaaataaaaacattaagttatgacgaagaagaacggaaacgccttaaaccggaaaattttcataaatagcgaaaacccgcgaggtcgccgccccgtaacaaggcggatcgccggaaaggacccgcaaatgataataattatcaattgcatactatcgacggcactgctgccagataacaccaccggggaaacattccatcatgatggccgtgcggacataggaagccagttcatccatcgctttcttgtctgctgccatttgctttgtgacatccagcgccgcacattcagcagcgtttttcagcgcgttttcgatcaacgtttcaatgttggtatcaacaccaggtttaactttgaacttatcggcactgacggttaccttgttctgcgctggctcatcacgctggataccaaggctgatgttgtagatattggtcaccggctgaggtgtttcgattgccgctgcgtggatagcaccatttgcgatagcggcgtccttgatgaatgacactccattgcgaataagttcgaaggagacggtgcccgggtctctc

SEQ ID NO: 10 - DNA, 689 bp, Artificial
  Molecule (B)
tccatgggcatactgatcggtagggcgcgttacctgtccgcctttctcccttcgggaagcgtggcgctttctcatagctcacgctgtaggtatctcagttcggtgtaggtcgttcgctccaagctgggctgtgtgcacgaaccccccgttcagcccgaccgctgcgccttatccggtaactatcgtcttgagtccaacccggtaagacacgacttatcgccactggcagcagccactggtaacaggattagcagagcgaggtatgtaggcggtgctacagagttcttgaagtggtggcctaactacggctacactagaaggacagtatttggtatctgcgctctgctgaagccagttaccttcggaaaaagagttggtagctcttgatccggcaaacaaaccaccgctggtagcggtggtttttttgtttgcaagcagcagattacgcgcagaaaaaaaggatctcaagaagatcctttgatcttttctacggggtctgacgctcagtggaacgaaaactcacgttaagggattttggtcatgagattatcaaaaaggatcttcacctagatccttttaaattaaaaatgaagttttaaatcaatctaaagtatatatgagtaaacttggtctgacagttaccaatgcttaatcagtgaggcctgcatggatggaggcgtcttggctca

SEQ ID NO: 11 - DNA, 62 bp, Artificial
  Oligo-TS1, Exemples 8 et 9
gagagacccgggcacgacttatcgccactggcagcagccactggtaacaggattagcagagc

SEQ ID NO: 12 - DNA, 26 bp, Artificial
  Oligo-L1, Exemples 8 et 9
tgagccaagacgcctccatccatgca

SEQ ID NO: 13 - DNA, 62 bp, Artificial
  Oligo-TS2, Exemples 8 et 9
gagagacccgggcaccgtctccttcgaacttattcgcaatggagtgtcattcatcaaggacg

SEQ ID NO: 14 - DNA, 25 bp, Artificial
  Oligo-L2, Exemples 8 et 9
tccatgggcatactgatcggtaggg

SEQ ID NO: 15 - DNA, 68 bp, Artificial
  Oligo-TS1, Exemple 10
atatgaggctgaggaagcggttagctccttcggtcctccgatcgttgtcagaagtaagttggccgcag

SEQ ID NO: 16 - DNA, 25 bp, Artificial
  Oligo-L1, Exemple 10
tccatgggcatactgatcggtaggg

SEQ ID NO: 17 - DNA, 59 bp, Artificial
  Oligo-TS2, Exemple 10
tgtaagagctgaggcggtgaccaatatctacaacatcagccttggtatccagcgtgatg

SEQ ID NO: 18 - DNA, 26 bp, Artificial
  Oligo-L2, Exemple 10
tgagccaagacgcctccatccatgca

SEQ ID NO: 19 - DNA, 38 bp, Artificial
  Oligo - forward pour amplication de la longe
gagagaacgcgttacctgtccgcctttctcccttcggg

SEQ ID NO: 20 - DNA, 47 bp, Artificial
  Oligo - reverse pour amplication de la longe
gagagacctgcaggcctcactgattaagcattggtaactgtcagacc

SEQ ID NO: 21 - DNA, 22 bp, Artificial
  Oligo-LC1, Exemples 8 et 9
tggatggaggcgtcttggctca

SEQ ID NO: 22 - DNA, 29 bp, Artificial
  Oligo-LC2, Exemples 8 et 9
cgcgccctaccgatcagtatgcccatgga

SEQ ID NO: 23 - DNA, 29 bp, Artificial
  Oligo-LC1, Exemple 10
cgcgccctaccgatcagtatgcccatgga

SEQ ID NO: 24 - DNA, 22 bp, Artificial
  Oligo-LC2, Exemple 10
tggatggaggcgtcttggctca

SEQ ID NO: 25 - DNA, 657 bp, Artificial
  Produit d'amplification pour utilisation en tant que longe
gagagaacgcgttacctgtccgcctttctcccttcgggaagcgtggcgctttctcatagctcacgctgtaggtatctcagttcggtgtaggtcgttcgctccaagctgggctgtgtgcacgaaccccccgttcagcccgaccgctgcgccttatccggtaactatcgtcttgagtccaacccggtaagacacgacttatcgccactggcagcagccactggtaacaggattagcagagcgaggtatgtaggcggtgctacagagttcttgaagtggtggcctaactacggctacactagaaggacagtatttggtatctgcgctctgctgaagccagttaccttcggaaaaagagttggtagctcttgatccggcaaacaaaccaccgctggtagcggtggtttttttgtttgcaagcagcagattacgcgcagaaaaaaaggatctcaagaagatcctttgatcttttctacggggtctgacgctcagtggaacgaaaactcacgttaagggattttggtcatgagattatcaaaaaggatcttcacctagatccttttaaattaaaaatgaagttttaaatcaatctaaagtatatatgagtaaacttggtctgacagttaccaatgcttaatcagtgaggcctgcaggtctctc

SEQ ID NO: 26 - DNA, 2853 bp, Artificial
  Molecule d'ADN double brin (1), variant (1.1), Exemples 8 et 9
gagagacccgggcacgacttatcgccactggcagcagccactggtaacaggattagcagagcgaggtatgtaggcggtgctacagagttcttgaagtggtggcctaactacggctacactagaaggacagtatttggtatctgcgctctgctgaagccagttaccttcggaaaaagagttggtagctcttgatccggcaaacaaaccaccgctggtagcggtggtttttttgtttgcaagcagcagattacgcgcagaaaaaaaggatctcaagaagatcctttgatcttttctacggggtctgacgctcagtggaacgaaaactcacgttaagggattttggtcatgagattatcaaaaaggatcttcacctagatccttttaaattaaaaatgaagttttaaatcaatctaaagtatatatgagtaaacttggtctgacagttaccaatgcttaatcagtgaggcacctatctcagcgatctgtctatttcgttcatcccatagttgcctgcaactccccgtcgtgtagataactacgatacgggagggcttaccatctggccccagtgctgcaatgataccgcgaagacccacgctcaccggctccagatttatcagcaataaaccagccagccggaagggccgagcgcagaagtggtcctgcaactttatccgcctccatccagtctattaattgttgccgggaagctagagtaagtagttcgccagttaatagtttgcgcaacgttgttgccattgctgcaggcatcgtggtgtcacgctcgtcgtttggtatggcttcattcagctccggttcccaacgatcaaggcgagttacatgatcccccatgttgtgcaaaaaagcggttagctccttcggtcctccgatcgttgtcagaagtaagttggccgcagtgttatcactcatggttatggcagcactgcataattctcttactgtcatgccatccgtaagatgcttttctgtgactggtgagtactcaaccaagtcattctgagaatagtgtatgcggcgaccgagttgctcttgcccggcgtcaacacgggataataccgcgccacatagcagaactttaaaagtgctcatcattggaaaacgttcttcggggcgaaaactctcaaggatcttaccgctgttgagatccagttcgatgtaacccactcgtgcacccaactgatcttcagcatcttttactttcaccagcgtttctgggtgagcaaaaacaggaaggcaaaatgccgcaaaaaagggaataagggcgacacggaaatgttgaatactcatactcttcctttttcaatattattgaagcatttatcagggttattgtctcatgagcggatacatatttgaatgtatttagaaaaataaacaaataggggttccgcgcacatttccccgaaaagtgccacctgacgtctaagaaaccattattatcatgacattaacctataaaaataggcgtatcacgaggccctttcgtcttcaagaattcgaattcgagctcttcatcatttcaagctattaaatattgctaacaggtatcgtttggaggcagggaagcacttgagtgaagtgattactcaaagaaactctttcgtaaaagttataaggaaatatagttcaaccgcaacgtttcagcagctacagtcagaatttattgaagcaaatctgaaacctattatagatttgaatgacttccccaattattggaaaagagttatgtatcagtgcctagcaaactcggaagattttttcagagggatctagaatatgatgaaagatagaaaattacgacgcttatcggaagtgaacgaatactttttatatgaggagggctgtttttacaaaatccggtagtaacttgctaaccaattcctaggcaggtcattggcaacagtggcatgcaccgagaaggacgtttgtaatgtccgctccggcacatagcagtcctagggacagtggcgtacagtcatagatggtcggtgggaggtggtacaaattctctcatgcaaaaaatatgtaaaatcggtagcaactggaaatcattcaacacccgcactatcggaagttcaccagccagccgcagcacgttcctgcatacgacgtgtctgcggctctaccatatctcctatgagcaacgtgttagcagagccaagccacaactctaattttaatacataatgaatgataataataatattaaaaatttcctgtgtaactaatttactatatggtttctgataagaatcattgcaaagatcaaacaacttgtattacattgacagttaagcagttaattttatcacctctaaaatatatcagcatctagcatgcaacctatcaaaatggagagttttatgactaaaaaaccatgggaaagaagacttaaagatttatcgcacttgctcaaatgctgcattgatacatattttgaccctgaattatttcgcttgaatttgaatcaattcctccaaaccgcaagaacagtaacatttattattcaaaaaaacaaaaaccagattataggatatgacatttggtataacaataatgttattgaaaaatggaaaaatgatccattaatggcttgggctaaaaattctcgcaatacgatagaaaaacaaggcgatttagaaatgtatagcgaggcaaaggctactcttatttcatcttacattgaagaaaatgacattgagtttattacaaatgaaagtatgttaaacattggtataaaaaagttagtcagacttgcacaaaagaaattaccttcatatttaactgaatcatctattattaaatcagaaagacgatgggtcgctaatacgc

SEQ ID NO: 27 - DNA, 2488 bp, Artificial
  Molecule d'ADN double brin (1), variant (1.2), Exemples 8 et 9
gagagacccgggcacgacttatcgccactggcagcagccactggtaacaggattagcagagcgaggtatgtaggcggtgctacagagttcttgaagtggtggcctaactacggctacactagaaggacagtatttggtatctgcgctctgctgaagccagttaccttcggaaaaagagttggtagctcttgatccggcaaacaaaccaccgctggtagcggtggtttttttgtttgcaagcagcagattacgcgcagaaaaaaaggatctcaagaagatcctttgatcttttctacggggtctgacgctcagtggaacgaaaactcacgttaagggattttggtcatgagattatcaaaaaggatcttcacctagatccttttaaattaaaaatgaagttttaaatcaatctaaagtatatatgagtaaacttggtctgacagttaccaatgcttaatcagtgaggcacctatctcagcgatctgtctatttcgttcatcccatagttgcctgcaactccccgtcgtgtagataactacgatacgggagggcttaccatctggccccagtgctgcaatgataccgcgaagacccacgctcaccggctccagatttatcagcaataaaccagccagccggaagggccgagcgcagaagtggtcctgcaactttatccgcctccatccagtctattaattgttgccgggaagctagagtaagtagttcgccagttaatagtttgcgcaacgttgttgccattgctgcaggcatcgtggtgtcacgctcgtcgtttggtatggcttcattcagctccggttcccaacgatcaaggcgagttacatgatcccccatgttgtgcaaaaaagcggttagctccttcggtcctccgatcgttgtcagaagtaagttggccgcagtgttatcactcatggttatggcagcactgcataattctcttactgtcatgccatccgtaagatgcttttctgtgactggtgagtactcaaccaagtcattctgagaatagtgtatgcggcgaccgagttgctcttgcccggcgtcaacacgggataataccgcgccacatagcagaactttaaaagtgctcatcattggaaaacgttcttcggggcgaaaactctcaaggatcttaccgctgttgagatccagttcgatgtaacccactcgtgcacccaactgatcttcagcatcttttactttcaccagcgtttctgggtgagcaaaaacaggaaggcaaaatgccgcaaaaaagggaataagggcgacacggaaatgttgaatactcatactcttcctttttcaatattattgaagcatttatcagggttattgtctcatgagcggatacatatttgaatgtatttagaaaaataaacaaataggggttccgcgcacatttccccgaaaagtgccacctgacgtctaagaaaccattattatcatgacattaacctataaaaataggcgtatcacgaggccctttcgtcttcaagaattcgaattcgagctctgtgtttgtcttcctgcctccagttcgccgggcattcaacataaaaactgatagcacccggagttccggaaacgaaatttgcatatacccattgctcacgaaaaaaaatgtccttgtcgatatagggatgaatcgcttggtgtacctcatctactgcgaaaacttgacctttctctcccatattgcagtcgcggcacgatggaactaaattaataggcatcaccgaaaattcaggataatgtgcaataggaagaaaatgatctatattttttgtctgtcctatatcaccacaaaatggacatttttcacctgatgaaacaagcatgtcatcgtaatatgttctagcgggtttgtttttatctcggagattattttcataaagcttttctaatttaacctttgtcaggttaccaactactaaggttgtaggctcaagagggtgtgtcctgtcgtaggtaaataactgacctgtcgagcttaatattctatattgttgttctttctgcaaaaaagtggggaagtgagtaatgaaattatttctaacatttatctgcatcataccttccgagcatttattaagcatttcgctataagttctcgctggaagaggtagttttttcattgtactttaccttcatctctgttcattatcatcgcttttaaaacggttcgaccttctaatcctatctgaccattataattttttagaatggtttcataagaaagctctgaatcaacggactgcgataataagtggtggtatccagaatttgtcacttcaagtaaaaacacctcacgagttaaaacacctaagttctcaccgaatgtctcaatatccggacggataatatttattgcttctcttgaccgtaggactttccacatgcaggattttggaacctcttgcagtactactggggaatgagttgcaattattgctacaccattgcgtgcatc

SEQ ID NO: 28 - DNA, 2552 bp, Artificial
  Molecule d'ADN double brin (2), variant (2.1), Exemples 8 et 9
gagagacccgggcaccgtctccttcgaacttattcgcaatggagtgtcattcatcaaggacgccgctatcgcaaatggtgctatccacgcagcggcaatcgaaacacctcagccggtgaccaatatctacaacatcagccttggtatccagcgtgatgagccagcgcagaacaaggtaaccgtcagtgccgataagttcaaagttaaacctggtgttgataccaacattgaaacgttgatcgaaaacgcgctgaaaaacgctgctgaatgtgcggcgctggatgtcacaaagcaaatggcagcagacaagaaagcgatggatgaactggcttcctatgtccgcacggccatcatgatggaatgtttccccggtggtgttatctggcagcagtgccgtcgatagtatgcaattgataattattatcatttgcgggtcctttccggcgatccgccttgttacggggcggcgacctcgcgggttttcgctatttatgaaaattttccggtttaaggcgtttccgttcttcttcgtcataacttaatgtttttatttaaaataccctctgaaaagaaaggaaacgacaggtgctgaaagcgagctttttggcctctgtcgtttcctttctctgtttttgtccgtggaatgaacaatggaagtcaacaaaaagcagctggctgacattttcggtgcgagtatccgtaccattcagaactggcaggaacagggaatgcccgttctgcgaggcggtggcaagggtaatgaggtgctttatgactctgccgccgtcataaaatggtatgccgaaagggatgctgaaattgagaacgaaaagctgcgccgggaggttgaagaactgcggcaggccaacgaggcagatccacaggacgggtgtggtcgccatgatcgcgtagtcgatagtggctccaagtagcgaagcgagcaggactgggcggcggccaaagcggtcggacagtgctccgagaacgggtgcgcatagaaattgcatcaacgcatatagcgctagcagcacgccatagtgactggcgatgctgtcggaatggacgatatcccgcaagaggcccggcagtaccggcataaccaagcctatgcctacagcatccagggtgacggtgccgaggatgacgatgagcgcattgttagatttcatacacggtgcctgactgcgttagcaatttaactgtgataaactaccgcattaaagcttgcatgcctgcatgcaggtcgacagtcagcagatgaacactgaccacaaggctgttttggataaggataatgcttatccagtggagtgctgggttcctgatccaagtaaaaatgaaaacactagatattttggaacctacacaggtggggaaaatgtgcctcctgttttgcacattactaacacagcaaccacagtgcttcttgatgagcagggtgttgggcccttgtgcaaagctgacagcttgtatgtttctgctgttgactctagaatatgatgaaagatagaaaattacgacgcttatcggaagtgaacgaatactttttatatgaggagggctgtttttacaaaatccggtagtaacttgctaaccaattcctaggcaggtcattggcaacagtggcatgcaccgagaaggacgtttgtaatgtccgctccggcacatagcagtcctagggacagtggcgtacagtcatagatggtcggtgggaggtggtacaaattctctcatgcaaaaaatatgtaaaatcggtagcaactggaaatcattcaacacccgcactatcggaagttcaccagccagccgcagcacgttcctgcatacgacgtgtctgcggctctaccatatctcctatgagcaacgtgttagcagagccaagccacaactctaattttaatacataatgaatgataataataatattaaaaatttcctgtgtaactaatttactatatggtttctgataagaatcattgcaaagatcaaacaacttgtattacattgacagttaagcagttaattttatcacctctaaaatatatcagcatctagcatgcaacctatcaaaatggagagttttatgactaaaaaaccatgggaaagaagacttaaagatttatcgcacttgctcaaatgctgcattgatacatattttgaccctgaattatttcgcttgaatttgaatcaattcctccaaaccgcaagaacagtaacatttattattcaaaaaaacaaaaaccagattataggatatgacatttggtataacaataatgttattgaaaaatggaaaaatgatccattaatggcttgggctaaaaattctcgcaatacgatagaaaaacaaggcgatttagaaatgtatagcgaggcaaaggctactcttatttcatcttacattgaagaaaatgacattgagtttattacaaatgaaagtatgttaaacattggtataaaaaagttagtcagacttgcacaaaagaaattaccttcatatttaactgaatcatctattattaaatcagaaagacgatgggtcgctaatacgc

SEQ ID NO: 29 - DNA, 2715 bp, Artificial
  Molecule d'ADN double brin (2), variant (2.2), Exemples 8 et 9
gagagacccgggcaccgtctccttcgaacttattcgcaatggagtgtcattcatcaaggacgccgctatcgcaaatggtgctatccacgcagcggcaatcgaaacacctcagccggtgaccaatatctacaacatcagccttggtatccagcgtgatgagccagcgcagaacaaggtaaccgtcagtgccgataagttcaaagttaaacctggtgttgataccaacattgaaacgttgatcgaaaacgcgctgaaaaacgctgctgaatgtgcggcgctggatgtcacaaagcaaatggcagcagacaagaaagcgatggatgaactggcttcctatgtccgcacggccatcatgatggaatgtttccccggtggtgttatctggcagcagtgccgtcgatagtatgcaattgataattattatcatttgcgggtcctttccggcgatccgccttgttacggggcggcgacctcgcgggttttcgctatttatgaaaattttccggtttaaggcgtttccgttcttcttcgtcataacttaatgtttttatttaaaataccctctgaaaagaaaggaaacgacaggtgctgaaagcgagctttttggcctctgtcgtttcctttctctgtttttgtccgtggaatgaacaatggaagtcaacaaaaagcagctggctgacattttcggtgcgagtatccgtaccattcagaactggcaggaacagggaatgcccgttctgcgaggcggtggcaagggtaatgaggtgctttatgactctgccgccgtcataaaatggtatgccgaaagggatgctgaaattgagaacgaaaagctgcgccgggaggttgaagaactgcggcaggccaacgaggcagatccacaggacgggtgtggtcgccatgatcgcgtagtcgatagtggctccaagtagcgaagcgagcaggactgggcggcggccaaagcggtcggacagtgctccgagaacgggtgcgcatagaaattgcatcaacgcatatagcgctagcagcacgccatagtgactggcgatgctgtcggaatggacgatatcccgcaagaggcccggcagtaccggcataaccaagcctatgcctacagcatccagggtgacggtgccgaggatgacgatgagcgcattgttagatttcatacacggtgcctgactgcgttagcaatttaactgtgataaactaccgcattaaagcttgcatgcctgcatgcaggtcgacagtcagcagatgaacactgaccacaaggctgttttggataaggataatgcttatccagtggagtgctgggttcctgatccaagtaaaaatgaaaacactagatattttggaacctacacaggtggggaaaatgtgcctcctgttttgcacattactaacacagcaaccacagtgcttcttgatgagcagggtgttgggcccttgtgcaaagctgacagcttgtatgtttctgctgttgactctagatccctctgaaaaaatcttccgagtttgctaggcactgatacataactcttttccaataattggggaagtcattcaaatctataataggtttcagatttgcttcaataaattctgactgtagctgctgaaacgttgcggttgaactatatttccttataacttttacgaaagagtttctttgagtaatcacttcactcaagtgcttccctgcctccaaacgatacctgttagcaatatttaatagcttgaaatgatgaagagctctgtgtttgtcttcctgcctccagttcgccgggcattcaacataaaaactgatagcacccggagttccggaaacgaaatttgcatatacccattgctcacgaaaaaaaatgtccttgtcgatatagggatgaatcgcttggtgtacctcatctactgcgaaaacttgacctttctctcccatattgcagtcgcggcacgatggaactaaattaataggcatcaccgaaaattcaggataatgtgcaataggaagaaaatgatctatattttttgtctgtcctatatcaccacaaaatggacatttttcacctgatgaaacaagcatgtcatcgtaatatgttctagcgggtttgtttttatctcggagattattttcataaagcttttctaatttaacctttgtcaggttaccaactactaaggttgtaggctcaagagggtgtgtcctgtcgtaggtaaataactgacctgtcgagcttaatattctatattgttgttctttctgcaaaaaagtggggaagtgagtaatgaaattatttctaacatttatctgcatcataccttccgagcatttattaagcatttcgctataagttctcgctggaagaggtagttttttcattgtactttaccttcatctctgttcattatcatcgcttttaaaacggttcgaccttctaatcctatctgaccattataattttttagaatggtttcataagaaagctctgaatcaacggactgcgataataagtggtggtatccagaatttgtcacttcaagtaaaaacacctcacgagttaaaacacctaagttctcaccgaatgtctcaatatccggacggataatatttattgcttctcttgaccgtaggactttccacatgcaggattttggaacctcttgcagtactactggggaatgagttgcaattattgctacaccattgcgtgcatc

SEQ ID NO: 30 - DNA, 2092 bp, Artificial
  Molecule (A), Exemple 10
atatgaggctgaggaagcggttagctccttcggtcctccgatcgttgtcagaagtaagttggccgcagtgttatcactcatggttatggcagcactgcataattctcttactgtcatgccatccgtaagatgcttttctgtgactggtgagtactcaaccaagtcattctgagaatagtgtatgcggcgaccgagttgctcttgcccggcgtcaacacgggataataccgcgccacatagcagaactttaaaagtgctcatcattggaaaacgttcttcggggcgaaaactctcaaggatcttaccgctgttgagatccagttcgatgtaacccactcgtgcacccaactgatcttcagcatcttttactttcaccagcgtttctgggtgagcaaaaacaggaaggcaaaatgccgcaaaaaagggaataagggcgacacggaaatgttgaatactcatactcttcctttttcaatattattgaagcatttatcagggttattgtctcatgagcggatacatatttgaatgtatttagaaaaataaacaaataggggttccgcgcacatttccccgaaaagtgccacctgacgtctaagaaaccattattatcatgacattaacctataaaaataggcgtatcacgaggccctttcgtcttcaagaattcgaattcgagctcggtacccggggatcctctagagtcaacagcagaaacatacaagctgtcagctttgcacaagggcccaacaccctgctcatcaagaagcactgtggttgctgtgttagtaatgtgcaaaacaggaggcacattttccccacctgtgtaggttccaaaatatctagtgttttcatttttacttggatcaggaacccagcactccactggataagcattatccttatccaaaacagccttgtggtcagtgttcatctgctgactgtcgacctgcatgcaggcatgcaagctttaatgcggtagtttatcacagttaaattgctaacgcagtcaggcaccgtgtatgaaatctaacaatgcgctcatcgtcatcctcggcaccgtcaccctggatgctgtaggcataggcttggttatgccggtactgccgggcctcttgcgggatatcgtccattccgacagcatcgccagtcactatggcgtgctgctagcgctatatgcgttgatgcaatttctatgcgcacccgttctcggagcactgtccgaccgctttggccgccgcccagtcctgctcgcttcgctacttggagccactatcgactacgcgatcatggcgaccacacccgtcctgtggatctgcctcgttggcctgccgcagttcttcaacctcccggcgcagcttttcgttctcaatttcagcatccctttcggcataccattttatgacggcggcagagtcataaagcacctcattacccttgccaccgcctcgcagaacgggcattccctgttcctgccagttctgaatggtacggatactcgcaccgaaaatgtcagccagctgctttttgttgacttccattgttcattccacggacaaaaacagagaaaggaaacgacagaggccaaaaagctcgctttcagcacctgtcgtttcctttcttttcagagggtattttaaataaaaacattaagttatgacgaagaagaacggaaacgccttaaaccggaaaattttcataaatagcgaaaacccgcgaggtcgccgccccgtaacaaggcggatcgccggaaaggacccgcaaatgataataattatcaattgcatactatcgacggcactgctgccagataacaccaccggggaaacattccatcatgatggccgtgcggacataggaagccagttcatccatcgctttcttgtctgctgccatttgctttgtgacatccagcgccgcacattcagcagcgtttttcagcgcgttttcgatcaacgtttcaatgttggtatcaacaccaggtttaactttgaacttatcggcactgacggttaccttgttctgcgctggctcatcacgctggataccaaggctgatgttgtagatattggtcaccgcctcagctcttaca

SEQ ID NO: 31 - DNA, 2005 bp, Artificial
  Molecule d'ADN double brin (1), variant (1.1), Exemple 10
tatatgaggctgaggaagcggttagctccttcggtcctccgatcgttgtcagaagtaagttggccgcagtgttatcactcatggttatggcagcactgcataattctcttactgtcatgccatccgtaagatgcttttctgtgactggtgagtactcaaccaagtcattctgagaatagtgtatgcggcgaccgagttgctcttgcccggcgtcaacacgggataataccgcgccacatagcagaactttaaaagtgctcatcattggaaaacgttcttcggggcgaaaactctcaaggatcttaccgctgttgagatccagttcgatgtaacccactcgtgcacccaactgatcttcagcatcttttactttcaccagcgtttctgggtgagcaaaaacaggaaggcaaaatgccgcaaaaaagggaataagggcgacacggaaatgttgaatactcatactcttcctttttcaatattattgaagcatttatcagggttattgtctcatgagcggatacatatttgaatgtatttagaaaaataaacaaataggggttccgcgcacatttccccgaaaagtgccacctgacgtctaagaaaccattattatcatgacattaacctataaaaataggcgtatcacgaggccctttcgtcttcaagaattcgaattcgagctcttcatcatttcaagctattaaatattgctaacaggtatcgtttggaggcagggaagcacttgagtgaagtgattactcaaagaaactctttcgtaaaagttataaggaaatatagttcaaccgcaacgtttcagcagctacagtcagaatttattgaagcaaatctgaaacctattatagatttgaatgacttccccaattattggaaaagagttatgtatcagtgcctagcaaactcggaagattttttcagagggatctagaatatgatgaaagatagaaaattacgacgcttatcggaagtgaacgaatactttttatatgaggagggctgtttttacaaaatccggtagtaacttgctaaccaattcctaggcaggtcattggcaacagtggcatgcaccgagaaggacgtttgtaatgtccgctccggcacatagcagtcctagggacagtggcgtacagtcatagatggtcggtgggaggtggtacaaattctctcatgcaaaaaatatgtaaaatcggtagcaactggaaatcattcaacacccgcactatcggaagttcaccagccagccgcagcacgttcctgcatacgacgtgtctgcggctctaccatatctcctatgagcaacgtgttagcagagccaagccacaactctaattttaatacataatgaatgataataataatattaaaaatttcctgtgtaactaatttactatatggtttctgataagaatcattgcaaagatcaaacaacttgtattacattgacagttaagcagttaattttatcacctctaaaatatatcagcatctagcatgcaacctatcaaaatggagagttttatgactaaaaaaccatgggaaagaagacttaaagatttatcgcacttgctcaaatgctgcattgatacatattttgaccctgaattatttcgcttgaatttgaatcaattcctccaaaccgcaagaacagtaacatttattattcaaaaaaacaaaaaccagattataggatatgacatttggtataacaataatgttattgaaaaatggaaaaatgatccattaatggcttgggctaaaaattctcgcaatacgatagaaaaacaaggcgatttagaaatgtatagcgaggcaaaggctactcttatttcatcttacattgaagaaaatgacattgagtttattacaaatgaaagtatgttaaacattggtataaaaaagttagtcagacttgcacaaaagaaattaccttcatatttaactgaatcatctattattaaatcagaaagacgatgggtcgctaatacgc

SEQ ID NO: 32 - DNA, 1640 bp, Artificial
  Molecule d'ADN double brin (1), variant (1.2), Exemple 10
tatatgaggctgaggaagcggttagctccttcggtcctccgatcgttgtcagaagtaagttggccgcagtgttatcactcatggttatggcagcactgcataattctcttactgtcatgccatccgtaagatgcttttctgtgactggtgagtactcaaccaagtcattctgagaatagtgtatgcggcgaccgagttgctcttgcccggcgtcaacacgggataataccgcgccacatagcagaactttaaaagtgctcatcattggaaaacgttcttcggggcgaaaactctcaaggatcttaccgctgttgagatccagttcgatgtaacccactcgtgcacccaactgatcttcagcatcttttactttcaccagcgtttctgggtgagcaaaaacaggaaggcaaaatgccgcaaaaaagggaataagggcgacacggaaatgttgaatactcatactcttcctttttcaatattattgaagcatttatcagggttattgtctcatgagcggatacatatttgaatgtatttagaaaaataaacaaataggggttccgcgcacatttccccgaaaagtgccacctgacgtctaagaaaccattattatcatgacattaacctataaaaataggcgtatcacgaggccctttcgtcttcaagaattcgaattcgagctctgtgtttgtcttcctgcctccagttcgccgggcattcaacataaaaactgatagcacccggagttccggaaacgaaatttgcatatacccattgctcacgaaaaaaaatgtccttgtcgatatagggatgaatcgcttggtgtacctcatctactgcgaaaacttgacctttctctcccatattgcagtcgcggcacgatggaactaaattaataggcatcaccgaaaattcaggataatgtgcaataggaagaaaatgatctatattttttgtctgtcctatatcaccacaaaatggacatttttcacctgatgaaacaagcatgtcatcgtaatatgttctagcgggtttgtttttatctcggagattattttcataaagcttttctaatttaacctttgtcaggttaccaactactaaggttgtaggctcaagagggtgtgtcctgtcgtaggtaaataactgacctgtcgagcttaatattctatattgttgttctttctgcaaaaaagtggggaagtgagtaatgaaattatttctaacatttatctgcatcataccttccgagcatttattaagcatttcgctataagttctcgctggaagaggtagttttttcattgtactttaccttcatctctgttcattatcatcgcttttaaaacggttcgaccttctaatcctatctgaccattataattttttagaatggtttcataagaaagctctgaatcaacggactgcgataataagtggtggtatccagaatttgtcacttcaagtaaaaacacctcacgagttaaaacacctaagttctcaccgaatgtctcaatatccggacggataatatttattgcttctcttgaccgtaggactttccacatgcaggattttggaacctcttgcagtactactggggaatgagttgcaattattgctacaccattgcgtgcatc

SEQ ID NO: 33 - DNA, 2453 bp, Artificial
  Molecule d'ADN double brin (2), variant (2.1), Exemple 10
tgtaagagctgaggcggtgaccaatatctacaacatcagccttggtatccagcgtgatgagccagcgcagaacaaggtaaccgtcagtgccgataagttcaaagttaaacctggtgttgataccaacattgaaacgttgatcgaaaacgcgctgaaaaacgctgctgaatgtgcggcgctggatgtcacaaagcaaatggcagcagacaagaaagcgatggatgaactggcttcctatgtccgcacggccatcatgatggaatgtttccccggtggtgttatctggcagcagtgccgtcgatagtatgcaattgataattattatcatttgcgggtcctttccggcgatccgccttgttacggggcggcgacctcgcgggttttcgctatttatgaaaattttccggtttaaggcgtttccgttcttcttcgtcataacttaatgtttttatttaaaataccctctgaaaagaaaggaaacgacaggtgctgaaagcgagctttttggcctctgtcgtttcctttctctgtttttgtccgtggaatgaacaatggaagtcaacaaaaagcagctggctgacattttcggtgcgagtatccgtaccattcagaactggcaggaacagggaatgcccgttctgcgaggcggtggcaagggtaatgaggtgctttatgactctgccgccgtcataaaatggtatgccgaaagggatgctgaaattgagaacgaaaagctgcgccgggaggttgaagaactgcggcaggccaacgaggcagatccacaggacgggtgtggtcgccatgatcgcgtagtcgatagtggctccaagtagcgaagcgagcaggactgggcggcggccaaagcggtcggacagtgctccgagaacgggtgcgcatagaaattgcatcaacgcatatagcgctagcagcacgccatagtgactggcgatgctgtcggaatggacgatatcccgcaagaggcccggcagtaccggcataaccaagcctatgcctacagcatccagggtgacggtgccgaggatgacgatgagcgcattgttagatttcatacacggtgcctgactgcgttagcaatttaactgtgataaactaccgcattaaagcttgcatgcctgcatgcaggtcgacagtcagcagatgaacactgaccacaaggctgttttggataaggataatgcttatccagtggagtgctgggttcctgatccaagtaaaaatgaaaacactagatattttggaacctacacaggtggggaaaatgtgcctcctgttttgcacattactaacacagcaaccacagtgcttcttgatgagcagggtgttgggcccttgtgcaaagctgacagcttgtatgtttctgctgttgactctagaatatgatgaaagatagaaaattacgacgcttatcggaagtgaacgaatactttttatatgaggagggctgtttttacaaaatccggtagtaacttgctaaccaattcctaggcaggtcattggcaacagtggcatgcaccgagaaggacgtttgtaatgtccgctccggcacatagcagtcctagggacagtggcgtacagtcatagatggtcggtgggaggtggtacaaattctctcatgcaaaaaatatgtaaaatcggtagcaactggaaatcattcaacacccgcactatcggaagttcaccagccagccgcagcacgttcctgcatacgacgtgtctgcggctctaccatatctcctatgagcaacgtgttagcagagccaagccacaactctaattttaatacataatgaatgataataataatattaaaaatttcctgtgtaactaatttactatatggtttctgataagaatcattgcaaagatcaaacaacttgtattacattgacagttaagcagttaattttatcacctctaaaatatatcagcatctagcatgcaacctatcaaaatggagagttttatgactaaaaaaccatgggaaagaagacttaaagatttatcgcacttgctcaaatgctgcattgatacatattttgaccctgaattatttcgcttgaatttgaatcaattcctccaaaccgcaagaacagtaacatttattattcaaaaaaacaaaaaccagattataggatatgacatttggtataacaataatgttattgaaaaatggaaaaatgatccattaatggcttgggctaaaaattctcgcaatacgatagaaaaacaaggcgatttagaaatgtatagcgaggcaaaggctactcttatttcatcttacattgaagaaaatgacattgagtttattacaaatgaaagtatgttaaacattggtataaaaaagttagtcagacttgcacaaaagaaattaccttcatatttaactgaatcatctattattaaatcagaaagacgatgggtcgctaatacgc

SEQ ID NO: 34 - DNA, 2616 bp, Artificial
  Molecule d'ADN double brin (2), variant (2.2), Exemple 10
tgtaagagctgaggcggtgaccaatatctacaacatcagccttggtatccagcgtgatgagccagcgcagaacaaggtaaccgtcagtgccgataagttcaaagttaaacctggtgttgataccaacattgaaacgttgatcgaaaacgcgctgaaaaacgctgctgaatgtgcggcgctggatgtcacaaagcaaatggcagcagacaagaaagcgatggatgaactggcttcctatgtccgcacggccatcatgatggaatgtttccccggtggtgttatctggcagcagtgccgtcgatagtatgcaattgataattattatcatttgcgggtcctttccggcgatccgccttgttacggggcggcgacctcgcgggttttcgctatttatgaaaattttccggtttaaggcgtttccgttcttcttcgtcataacttaatgtttttatttaaaataccctctgaaaagaaaggaaacgacaggtgctgaaagcgagctttttggcctctgtcgtttcctttctctgtttttgtccgtggaatgaacaatggaagtcaacaaaaagcagctggctgacattttcggtgcgagtatccgtaccattcagaactggcaggaacagggaatgcccgttctgcgaggcggtggcaagggtaatgaggtgctttatgactctgccgccgtcataaaatggtatgccgaaagggatgctgaaattgagaacgaaaagctgcgccgggaggttgaagaactgcggcaggccaacgaggcagatccacaggacgggtgtggtcgccatgatcgcgtagtcgatagtggctccaagtagcgaagcgagcaggactgggcggcggccaaagcggtcggacagtgctccgagaacgggtgcgcatagaaattgcatcaacgcatatagcgctagcagcacgccatagtgactggcgatgctgtcggaatggacgatatcccgcaagaggcccggcagtaccggcataaccaagcctatgcctacagcatccagggtgacggtgccgaggatgacgatgagcgcattgttagatttcatacacggtgcctgactgcgttagcaatttaactgtgataaactaccgcattaaagcttgcatgcctgcatgcaggtcgacagtcagcagatgaacactgaccacaaggctgttttggataaggataatgcttatccagtggagtgctgggttcctgatccaagtaaaaatgaaaacactagatattttggaacctacacaggtggggaaaatgtgcctcctgttttgcacattactaacacagcaaccacagtgcttcttgatgagcagggtgttgggcccttgtgcaaagctgacagcttgtatgtttctgctgttgactctagatccctctgaaaaaatcttccgagtttgctaggcactgatacataactcttttccaataattggggaagtcattcaaatctataataggtttcagatttgcttcaataaattctgactgtagctgctgaaacgttgcggttgaactatatttccttataacttttacgaaagagtttctttgagtaatcacttcactcaagtgcttccctgcctccaaacgatacctgttagcaatatttaatagcttgaaatgatgaagagctctgtgtttgtcttcctgcctccagttcgccgggcattcaacataaaaactgatagcacccggagttccggaaacgaaatttgcatatacccattgctcacgaaaaaaaatgtccttgtcgatatagggatgaatcgcttggtgtacctcatctactgcgaaaacttgacctttctctcccatattgcagtcgcggcacgatggaactaaattaataggcatcaccgaaaattcaggataatgtgcaataggaagaaaatgatctatattttttgtctgtcctatatcaccacaaaatggacatttttcacctgatgaaacaagcatgtcatcgtaatatgttctagcgggtttgtttttatctcggagattattttcataaagcttttctaatttaacctttgtcaggttaccaactactaaggttgtaggctcaagagggtgtgtcctgtcgtaggtaaataactgacctgtcgagcttaatattctatattgttgttctttctgcaaaaaagtggggaagtgagtaatgaaattatttctaacatttatctgcatcataccttccgagcatttattaagcatttcgctataagttctcgctggaagaggtagttttttcattgtactttaccttcatctctgttcattatcatcgcttttaaaacggttcgaccttctaatcctatctgaccattataattttttagaatggtttcataagaaagctctgaatcaacggactgcgataataagtggtggtatccagaatttgtcacttcaagtaaaaacacctcacgagttaaaacacctaagttctcaccgaatgtctcaatatccggacggataatatttattgcttctcttgaccgtaggactttccacatgcaggattttggaacctcttgcagtactactggggaatgagttgcaattattgctacaccattgcgtgcatc

SEQ ID NO: 35 - protein, 314 aa, Artificial
  Séquence 10xHis-SNAP-FRB
MGHHHHHHHHHHSSGMDKDCEMKRTTLDSPLGKLELSGCEQGLHEIKLLGKGTSAADAVEVPAPAAVLGGPEPLMQATAWLNAYFHQPEAIEEFPVPALHHPVFQQESFTRQVLWKLLKVVKFGEVISYQQLAALAGNPAATAAVKTALSGNPVPILIPCHRVVSSSGAVGGYEGGLAVKEWLLAHEGHRLGKPGLGSSGKLLEVLFQGPSSGELAILWHEMWHEGLEEASRLYFGERNVKGMFEVLEPLHAMMERGPQTLKETSFNQAYGRDLMEAQEWCRKYMKSGNVKDLTQAWDLYYHVFRRISKQLPQL

SEQ ID NO: 36 - protein, 323 aa, Artificial
  Séquence 10xHis-CLIP-FKBP12
MGHHHHHHHHHHSSGMDKDCEMKRTTLDSPLGKLELSGCEQGLHRIIFLGKGTSAADAVEVPAPAAVLGGPEPLIQATAWLNAYFHQPEAIEEFPVPALHHPVFQQESFTRQVLWKLLKVVKFGEVISESHLAALVGNPAATAAVNTALDGNPVPILIPCHRVVQGDSDVGPYLGGLAVKEWLLAHEGHRLGKPGLGSSGKLLEVLFQGPSSGELMGVQVETISPGDGRTFPKRGQTCVVHYTGMLEDGKKFDSSRDRNKPFKFMLGKQEVIRGWEEGVAQMSVGQRAKLTISPDYAYGATGHPGIIPPHATLVFDVELLKLE

SEQ ID NO: 37 - protein, 454 aa, Artificial
  Séquence 10xHis_CLIP_PHloop
MGHHHHHHHHHHSSGMDKDCEMKRTTLDSPLGKLELSGCEQGLHRIIFLGKGTSAADAVEVPAPAAVLGGPEPLIQATAWLNAYFHQPEAIEEFPVPALHHPVFQQESFTRQVLWKLLKVVKFGEVISESHLAALVGNPAATAAVNTALDGNPVPILIPCHRVVQGDSDVGPYLGGLAVKEWLLAHEGHRLGKPGLGSSGKLLEVLFQGPSSGELMANPDREGWLLKLGGGRVKTWKRRWFILTDNALYYFEYTTDKEPRGIIPLENLSIREVEDSKKPNVFELYIPDNKDQVIKAAKTEAKRVEAEKARIAKAEQADGKGGNAAKKNTVNGTGTPVHISTLQVGETRCKKVCTSKSDLRSNDFSIVGSLPRDFELSNYDCYGKPIEVNNGLGKPQAKNKKPPPAKPVIPTAAKRIDLYARVDGNHTVYRISAPTPEEKEEWIKAIKAAISRDG

SEQ ID NO: 38 - protein, 968 aa, Artificial
  Séquence 6xHis_SNAP_GephyrinrC4
MRGSHHHHHHGSACELSSGLEVLFQGPHMASMDKDCEMKRTTLDSPLGKLELSGCEQGLHEIKLLGKGTSAADAVEVPAPAAVLGGPEPLMQATAWLNAYFHQPEAIEEFPVPALHHPVFQQESFTRQVLWKLLKVVKFGEVISYQQLAALAGNPAATAAVKTALSGNPVPILIPCHRVVSSSGAVGGYEGGLAVKEWLLAHEGHRLGKPGLGSSGGTMATEGMILTNHDHQIRVGVLTVSDSCFRNLAEDRSGINLKDLVQDPSLLGGTISAYKIVPDEIEEIKETLIDWCDEKELNLILTTGGTGFAPRDVTPEATKEVIEREAPGMALAMLMGSLNVTPLGMLSRPVCGIRGKTLIINLPGSKKGSQECFQFILPALPHAIDLLRDAIVKVKEVHDELEDLPSPPPPLSPPPTTSPHKQTEDKGVQCEEEEEEKKDSGVASTEDSSSSHITAAALAAKIPDSIISRGVQVLPRDTASLSTTPSESPRAQATSRLSTASCPTPKARLPSCSSTYSVSEVQSRCSSKENILRASHSAVDITKVARRHRMSPFPLTSMDKAFITVLEMTPVLGTEIINYRDGMGRVLAQDVYAKDNLPPFPASVKDGYAVRAADGPGDRFIIGESQAGEQPTQTVMPGQVMRVTTGAPIPCGADAVVQVEDTELIRESDDGTEELEVRILVQARPGQDIRPIGHDIKRGECVLAKGTHMGPSEIGLLATVGVTEVEVNKFPVVAVMSTGNELLNPEDDLLPGKIRDSNRSTLLATIQEHGYPTINLGIVGDNPDDLLNALNEGISRADVIITSGGVSMGEKDYLKQVLDIDLHAQIHFGRVFMKPGLPTTFATLDIDGVRKIIFALPGNPVSAVVTCNLFVVPALRKMQGILDPRPTIIKARLSCDVKLDPRPEYHRCILTWHHQEPLPWAQSTGNQMSSRLMSMRSANGLLMLPPKTEQYVELHKGEVVDVMVIGRL

SEQ ID NO: 39 - DNA, 58 bp, Artificial
  Oligo-TS1  avec un O2-benzylcytosine-dT au bout 5'
gtaagagctgaggcggtgaccaatatctacaacatcagccttggtatccagcgtgatg

SEQ ID NO: 40 - DNA, 67 bp, Artificial
  Oligo-TS2 avec un O6-benzylguanine-dA au bout 5'
tctcaagctgaggaagcggttagctccttcggtcctccgatcgttgtcagaagtaagttggccgcag

SEQ ID NO: 41 - DNA, 42 bp, Artificial
  Oligonucleotide pour amplification de la matrice lambda par PCR
gagagaacgcgttccggatgcggagtcttatccgtggaaatc

SEQ ID NO: 42 - DNA, 44 bp, Artificial
  Oligonucleotide pour amplification de la matrice lambda par PCR
gagagacctgcaggaccagagcggagataatcgcggtgactctg

SEQ ID NO: 43 - DNA, 6058 bp, Artificial
  Longe d'environ 6 kbp, obtenu à partir de l'ADN  de la matrice phage lambda
tccatgggcatactgatcggtagggcgcgttccggatgcggagtcttatccgtggaaatcaaacgcgcactactggctggttaccaacctgtatcagaacatgcgggccaatgcgcttactgatgcggaattacgccgtaaggccgcagatgagcttgtccatatgactgcgagaattaaccgtggtgaggcgatccctgaaccagtaaaacaacttcctgtcatgggcggtagacctctaaatcgtgcacaggctctggcgaagatcgcagaaatcaaagctaagttcggactgaaaggagcaagtgtatgacgggcaaagaggcaattattcattacctggggacgcataatagcttctgtgcgccggacgttgccgcgctaacaggcgcaacagtaaccagcataaatcaggccgcggctaaaatggcacgggcaggtcttctggttatcgaaggtaaggtctggcgaacggtgtattaccggtttgctaccagggaagaacgggaaggaaagatgagcacgaacctggtttttaaggagtgtcgccagagtgccgcgatgaaacgggtattggcggtatatggagttaaaagatgaccatctacattactgagctaataacaggcctgctggtaatcgcaggcctttttatttgggggagagggaagtcatgaaaaaactaacctttgaaattcgatctccagcacatcagcaaaacgctattcacgcagtacagcaaatccttccagacccaaccaaaccaatcgtagtaaccattcaggaacgcaaccgcagcttagaccaaaacaggaagctatgggcctgcttaggtgacgtctctcgtcaggttgaatggcatggtcgctggctggatgcagaaagctggaagtgtgtgtttaccgcagcattaaagcagcaggatgttgttcctaaccttgccgggaatggctttgtggtaataggccagtcaaccagcaggatgcgtgtaggcgaatttgcggagctattagagcttatacaggcattcggtacagagcgtggcgttaagtggtcagacgaagcgagactggctctggagtggaaagcgagatggggagacagggctgcatgataaatgtcgttagtttctccggtggcaggacgtcagcatatttgctctggctaatggagcaaaagcgacgggcaggtaaagacgtgcattacgttttcatggatacaggttgtgaacatccaatgacatatcggtttgtcagggaagttgtgaagttctgggatataccgctcaccgtattgcaggttgatatcaacccggagcttggacagccaaatggttatacggtatgggaaccaaaggatattcagacgcgaatgcctgttctgaagccatttatcgatatggtaaagaaatatggcactccatacgtcggcggcgcgttctgcactgacagattaaaactcgttcccttcaccaaatactgtgatgaccatttcgggcgagggaattacaccacgtggattggcatcagagctgatgaaccgaagcggctaaagccaaagcctggaatcagatatcttgctgaactgtcagactttgagaaggaagatatcctcgcatggtggaagcaacaaccattcgatttgcaaataccggaacatctcggtaactgcatattctgcattaaaaaatcaacgcaaaaaatcggacttgcctgcaaagatgaggagggattgcagcgtgtttttaatgaggtcatcacgggatcccatgtgcgtgacggacatcgggaaacgccaaaggagattatgtaccgaggaagaatgtcgctggacggtatcgcgaaaatgtattcagaaaatgattatcaagccctgtatcaggacatggtacgagctaaaagattcgataccggctcttgttctgagtcatgcgaaatatttggagggcagcttgatttcgacttcgggagggaagctgcatgatgcgatgttatcggtgcggtgaatgcaaagaagataaccgcttccgaccaaatcaaccttactggaatcgatggtgtctccggtgtgaaagaacaccaacaggggtgttaccactaccgcaggaaaaggaggacgtgtggcgagacagcgacgaagtatcaccgacataatctgcgaaaactgcaaataccttccaacgaaacgcaccagaaataaacccaagccaatcccaaaagaatctgacgtaaaaaccttcaactacacggctcacctgtgggatatccggtggctaagacgtcgtgcgaggaaaacaaggtgattgaccaaaatcgaagttacgaacaagaaagcgtcgagcgagctttaacgtgcgctaactgcggtcagaagctgcatgtgctggaagttcacgtgtgtgagcactgctgcgcagaactgatgagcgatccgaatagctcgatgcacgaggaagaagatgatggctaaaccagcgcgaagacgatgtaaaaacgatgaatgccgggaatggtttcaccctgcattcgctaatcagtggtggtgctctccagagtgtggaaccaagatagcactcgaacgacgaagtaaagaacgcgaaaaagcggaaaaagcagcagagaagaaacgacgacgagaggagcagaaacagaaagataaacttaagattcgaaaactcgccttaaagccccgcagttactggattaaacaagcccaacaagccgtaaacgccttcatcagagaaagagaccgcgacttaccatgtatctcgtgcggaacgctcacgtctgctcagtgggatgccggacattaccggacaactgctgcggcacctcaactccgatttaatgaacgcaatattcacaagcaatgcgtggtgtgcaaccagcacaaaagcggaaatctcgttccgtatcgcgtcgaactgattagccgcatcgggcaggaagcagtagacgaaatcgaatcaaaccataaccgccatcgctggactatcgaagagtgcaaggcgatcaaggcagagtaccaacagaaactcaaagacctgcgaaatagcagaagtgaggccgcatgacgttctcagtaaaaaccattccagacatgctcgttgaagcatacggaaatcagacagaagtagcacgcagactgaaatgtagtcgcggtacggtcagaaaatacgttgatgataaagacgggaaaatgcacgccatcgtcaacgacgttctcatggttcatcgcggatggagtgaaagagatgcgctattacgaaaaaattgatggcagcaaataccgaaatatttgggtagttggcgatctgcacggatgctacacgaacctgatgaacaaactggatacgattggattcgacaacaaaaaagacctgcttatctcggtgggcgatttggttgatcgtggtgcagagaacgttgaatgcctggaattaatcacattcccctggttcagagctgtacgtggaaaccatgagcaaatgatgattgatggcttatcagagcgtggaaacgttaatcactggctgcttaatggcggtggctggttctttaatctcgattacgacaaagaaattctggctaaagctcttgcccataaagcagatgaacttccgttaatcatcgaactggtgagcaaagataaaaaatatgttatctgccacgccgattatccctttgacgaatacgagtttggaaagccagttgatcatcagcaggtaatctggaaccgcgaacgaatcagcaactcacaaaacgggatcgtgaaagaaatcaaaggcgcggacacgttcatctttggtcatacgccagcagtgaaaccactcaagtttgccaaccaaatgtatatcgataccggcgcagtgttctgcggaaacctaacattgattcaggtacagggagaaggcgcatgagactcgaaagcgtagctaaatttcattcgccaaaaagcccgatgatgagcgactcaccacgggccacggcttctgactctctttccggtactgatgtgatggctgctatggggatggcgcaatcacaagccggattcggtatggctgcattctgcggtaagcacgaactcagccagaacgacaaacaaaaggctatcaactatctgatgcaatttgcacacaaggtatcggggaaataccgtggtgtggcaaagcttgaaggaaatactaaggcaaaggtactgcaagtgctcgcaacattcgcttatgcggattattgccgtagtgccgcgacgccgggggcaagatgcagagattgccatggtacaggccgtgcggttgatattgccaaaacagagctgtgggggagagttgtcgagaaagagtgcggaagatgcaaaggcgtcggctattcaaggatgccagcaagcgcagcatatcgcgctgtgacgatgctaatcccaaaccttacccaacccacctggtcacgcactgttaagccgctgtatgacgctctggtggtgcaatgccacaaagaagagtcaatcgcagacaacattttgaatgcggtcacacgttagcagcatgattgccacggatggcaacatattaacggcatgatattgacttattgaataaaattgggtaaatttgactcaacgatgggttaattcgctcgttgtggtagtgagatgaaaagaggcggcgcttactaccgattccgcctagttggtcacttcgacgtatcgtctggaactccaaccatcgcaggcagagaggtctgcaaaatgcaatcccgaaacagttcgcaggtaatagttagagcctgcataacggtttcgggattttttatatctgcacaacaggtaagagcattgagtcgataatcgtgaagagtcggcgagcctggttagccagtgctctttccgttgtgctgaattaagcgaataccggaagcagaaccggatcaccaaatgcgtacaggcgtcatcgccgcccagcaacagcacaacccaaactgagccgtagccactgtctgtcctgaattcattagtaatagttacgctgcggccttttacacatgaccttcgtgaaagcgggtggcaggaggtcgcgctaacaacctcctgccgttttgcccgtgcatatcggtcacgaacaaatctgattactaaacacagtagcctggatttgttctatcagtaatcgaccttattcctaattaaatagagcaaatccccttattgggggtaagacatgaagatgccagaaaaacatgacctgttggccgccattctcgcggcaaaggaacaaggcatcggggcaatccttgcgtttgcaatggcgtaccttcgcggcagatataatggcggtgcgtttacaaaaacagtaatcgacgcaacgatgtgcgccattatcgcctggttcattcgtgaccttctcgacttcgccggactaagtagcaatctcgcttatataacgagcgtgtttatcggctacatcggtactgactcgattggttcgcttatcaaacgcttcgctgctaaaaaagccggagtagaagatggtagaaatcaataatcaacgtaaggcgttcctcgatatgctggcgtggtcggagggaactgataacggacgtcagaaaaccagaaatcatggttatgacgtcattgtaggcggagagctatttactgattactccgatcaccctcgcaaacttgtcacgctaaacccaaaactcaaatcaacaggcgccggacgctaccagcttctttcccgttggtgggatgcctaccgcaagcagcttggcctgaaagacttctctccgaaaagtcaggacgctgtggcattgcagcagattaaggagcgtggcgctttacctatgattgatcgtggtgatatccgtcaggcaatcgaccgttgcagcaatatctgggcttcactgccgggcgctggttatggtcagttcgagcataaggctgacagcctgattgcaaaattcaaagaagcgggcggaacggtcagagagattgatgtatgagcagagtcaccgcgattatctccgctctggtcctgcatggatggaggcgtcttggctca

SEQ ID NO: 44 - protein, 239 aa, Artificial
  PH-Loop
MANPDREGWLLKLGGGRVKTWKRRWFILTDNALYYFEYTTDKEPRGIIPLENLSIREVEDSKKPNVFELYIPDNKDQVIKAAKTEAKRVEAEKARIAKAEQADGKGGNAAKKNTVNGTGTPVHISTLQVGETRCKKVCTSKSDLRSNDFSIVGSLPRDFELSNYDCYGKPIEVNNGLGKPQAKNKKPPPAKPVIPTAAKRIDLYARVDGNHTVYRISAPTPEEKEEWIKAIKAAISRDG

SEQ ID NO: 45 - DNA, 2091 bp, Artificial
  Molécule (A), Exemple 12
tctcaagctgaggaagcggttagctccttcggtcctccgatcgttgtcagaagtaagttggccgcagtgttatcactcatggttatggcagcactgcataattctcttactgtcatgccatccgtaagatgcttttctgtgactggtgagtactcaaccaagtcattctgagaatagtgtatgcggcgaccgagttgctcttgcccggcgtcaacacgggataataccgcgccacatagcagaactttaaaagtgctcatcattggaaaacgttcttcggggcgaaaactctcaaggatcttaccgctgttgagatccagttcgatgtaacccactcgtgcacccaactgatcttcagcatcttttactttcaccagcgtttctgggtgagcaaaaacaggaaggcaaaatgccgcaaaaaagggaataagggcgacacggaaatgttgaatactcatactcttcctttttcaatattattgaagcatttatcagggttattgtctcatgagcggatacatatttgaatgtatttagaaaaataaacaaataggggttccgcgcacatttccccgaaaagtgccacctgacgtctaagaaaccattattatcatgacattaacctataaaaataggcgtatcacgaggccctttcgtcttcaagaattcgaattcgagctcggtacccggggatcctctagagtcaacagcagaaacatacaagctgtcagctttgcacaagggcccaacaccctgctcatcaagaagcactgtggttgctgtgttagtaatgtgcaaaacaggaggcacattttccccacctgtgtaggttccaaaatatctagtgttttcatttttacttggatcaggaacccagcactccactggataagcattatccttatccaaaacagccttgtggtcagtgttcatctgctgactgtcgacctgcatgcaggcatgcaagctttaatgcggtagtttatcacagttaaattgctaacgcagtcaggcaccgtgtatgaaatctaacaatgcgctcatcgtcatcctcggcaccgtcaccctggatgctgtaggcataggcttggttatgccggtactgccgggcctcttgcgggatatcgtccattccgacagcatcgccagtcactatggcgtgctgctagcgctatatgcgttgatgcaatttctatgcgcacccgttctcggagcactgtccgaccgctttggccgccgcccagtcctgctcgcttcgctacttggagccactatcgactacgcgatcatggcgaccacacccgtcctgtggatctgcctcgttggcctgccgcagttcttcaacctcccggcgcagcttttcgttctcaatttcagcatccctttcggcataccattttatgacggcggcagagtcataaagcacctcattacccttgccaccgcctcgcagaacgggcattccctgttcctgccagttctgaatggtacggatactcgcaccgaaaatgtcagccagctgctttttgttgacttccattgttcattccacggacaaaaacagagaaaggaaacgacagaggccaaaaagctcgctttcagcacctgtcgtttcctttcttttcagagggtattttaaataaaaacattaagttatgacgaagaagaacggaaacgccttaaaccggaaaattttcataaatagcgaaaacccgcgaggtcgccgccccgtaacaaggcggatcgccggaaaggacccgcaaatgataataattatcaattgcatactatcgacggcactgctgccagataacaccaccggggaaacattccatcatgatggccgtgcggacataggaagccagttcatccatcgctttcttgtctgctgccatttgctttgtgacatccagcgccgcacattcagcagcgtttttcagcgcgttttcgatcaacgtttcaatgttggtatcaacaccaggtttaactttgaacttatcggcactgacggttaccttgttctgcgctggctcatcacgctggataccaaggctgatgttgtagatattggtcaccgcctcagctcttaca

SEQ ID NO: 46 - DNA, 6011 bp, Artificial
  Produit de digestion  qui sera utilisé en tant que longe (6kbp)
cgcgttccggatgcggagtcttatccgtggaaatcaaacgcgcactactggctggttaccaacctgtatcagaacatgcgggccaatgcgcttactgatgcggaattacgccgtaaggccgcagatgagcttgtccatatgactgcgagaattaaccgtggtgaggcgatccctgaaccagtaaaacaacttcctgtcatgggcggtagacctctaaatcgtgcacaggctctggcgaagatcgcagaaatcaaagctaagttcggactgaaaggagcaagtgtatgacgggcaaagaggcaattattcattacctggggacgcataatagcttctgtgcgccggacgttgccgcgctaacaggcgcaacagtaaccagcataaatcaggccgcggctaaaatggcacgggcaggtcttctggttatcgaaggtaaggtctggcgaacggtgtattaccggtttgctaccagggaagaacgggaaggaaagatgagcacgaacctggtttttaaggagtgtcgccagagtgccgcgatgaaacgggtattggcggtatatggagttaaaagatgaccatctacattactgagctaataacaggcctgctggtaatcgcaggcctttttatttgggggagagggaagtcatgaaaaaactaacctttgaaattcgatctccagcacatcagcaaaacgctattcacgcagtacagcaaatccttccagacccaaccaaaccaatcgtagtaaccattcaggaacgcaaccgcagcttagaccaaaacaggaagctatgggcctgcttaggtgacgtctctcgtcaggttgaatggcatggtcgctggctggatgcagaaagctggaagtgtgtgtttaccgcagcattaaagcagcaggatgttgttcctaaccttgccgggaatggctttgtggtaataggccagtcaaccagcaggatgcgtgtaggcgaatttgcggagctattagagcttatacaggcattcggtacagagcgtggcgttaagtggtcagacgaagcgagactggctctggagtggaaagcgagatggggagacagggctgcatgataaatgtcgttagtttctccggtggcaggacgtcagcatatttgctctggctaatggagcaaaagcgacgggcaggtaaagacgtgcattacgttttcatggatacaggttgtgaacatccaatgacatatcggtttgtcagggaagttgtgaagttctgggatataccgctcaccgtattgcaggttgatatcaacccggagcttggacagccaaatggttatacggtatgggaaccaaaggatattcagacgcgaatgcctgttctgaagccatttatcgatatggtaaagaaatatggcactccatacgtcggcggcgcgttctgcactgacagattaaaactcgttcccttcaccaaatactgtgatgaccatttcgggcgagggaattacaccacgtggattggcatcagagctgatgaaccgaagcggctaaagccaaagcctggaatcagatatcttgctgaactgtcagactttgagaaggaagatatcctcgcatggtggaagcaacaaccattcgatttgcaaataccggaacatctcggtaactgcatattctgcattaaaaaatcaacgcaaaaaatcggacttgcctgcaaagatgaggagggattgcagcgtgtttttaatgaggtcatcacgggatcccatgtgcgtgacggacatcgggaaacgccaaaggagattatgtaccgaggaagaatgtcgctggacggtatcgcgaaaatgtattcagaaaatgattatcaagccctgtatcaggacatggtacgagctaaaagattcgataccggctcttgttctgagtcatgcgaaatatttggagggcagcttgatttcgacttcgggagggaagctgcatgatgcgatgttatcggtgcggtgaatgcaaagaagataaccgcttccgaccaaatcaaccttactggaatcgatggtgtctccggtgtgaaagaacaccaacaggggtgttaccactaccgcaggaaaaggaggacgtgtggcgagacagcgacgaagtatcaccgacataatctgcgaaaactgcaaataccttccaacgaaacgcaccagaaataaacccaagccaatcccaaaagaatctgacgtaaaaaccttcaactacacggctcacctgtgggatatccggtggctaagacgtcgtgcgaggaaaacaaggtgattgaccaaaatcgaagttacgaacaagaaagcgtcgagcgagctttaacgtgcgctaactgcggtcagaagctgcatgtgctggaagttcacgtgtgtgagcactgctgcgcagaactgatgagcgatccgaatagctcgatgcacgaggaagaagatgatggctaaaccagcgcgaagacgatgtaaaaacgatgaatgccgggaatggtttcaccctgcattcgctaatcagtggtggtgctctccagagtgtggaaccaagatagcactcgaacgacgaagtaaagaacgcgaaaaagcggaaaaagcagcagagaagaaacgacgacgagaggagcagaaacagaaagataaacttaagattcgaaaactcgccttaaagccccgcagttactggattaaacaagcccaacaagccgtaaacgccttcatcagagaaagagaccgcgacttaccatgtatctcgtgcggaacgctcacgtctgctcagtgggatgccggacattaccggacaactgctgcggcacctcaactccgatttaatgaacgcaatattcacaagcaatgcgtggtgtgcaaccagcacaaaagcggaaatctcgttccgtatcgcgtcgaactgattagccgcatcgggcaggaagcagtagacgaaatcgaatcaaaccataaccgccatcgctggactatcgaagagtgcaaggcgatcaaggcagagtaccaacagaaactcaaagacctgcgaaatagcagaagtgaggccgcatgacgttctcagtaaaaaccattccagacatgctcgttgaagcatacggaaatcagacagaagtagcacgcagactgaaatgtagtcgcggtacggtcagaaaatacgttgatgataaagacgggaaaatgcacgccatcgtcaacgacgttctcatggttcatcgcggatggagtgaaagagatgcgctattacgaaaaaattgatggcagcaaataccgaaatatttgggtagttggcgatctgcacggatgctacacgaacctgatgaacaaactggatacgattggattcgacaacaaaaaagacctgcttatctcggtgggcgatttggttgatcgtggtgcagagaacgttgaatgcctggaattaatcacattcccctggttcagagctgtacgtggaaaccatgagcaaatgatgattgatggcttatcagagcgtggaaacgttaatcactggctgcttaatggcggtggctggttctttaatctcgattacgacaaagaaattctggctaaagctcttgcccataaagcagatgaacttccgttaatcatcgaactggtgagcaaagataaaaaatatgttatctgccacgccgattatccctttgacgaatacgagtttggaaagccagttgatcatcagcaggtaatctggaaccgcgaacgaatcagcaactcacaaaacgggatcgtgaaagaaatcaaaggcgcggacacgttcatctttggtcatacgccagcagtgaaaccactcaagtttgccaaccaaatgtatatcgataccggcgcagtgttctgcggaaacctaacattgattcaggtacagggagaaggcgcatgagactcgaaagcgtagctaaatttcattcgccaaaaagcccgatgatgagcgactcaccacgggccacggcttctgactctctttccggtactgatgtgatggctgctatggggatggcgcaatcacaagccggattcggtatggctgcattctgcggtaagcacgaactcagccagaacgacaaacaaaaggctatcaactatctgatgcaatttgcacacaaggtatcggggaaataccgtggtgtggcaaagcttgaaggaaatactaaggcaaaggtactgcaagtgctcgcaacattcgcttatgcggattattgccgtagtgccgcgacgccgggggcaagatgcagagattgccatggtacaggccgtgcggttgatattgccaaaacagagctgtgggggagagttgtcgagaaagagtgcggaagatgcaaaggcgtcggctattcaaggatgccagcaagcgcagcatatcgcgctgtgacgatgctaatcccaaaccttacccaacccacctggtcacgcactgttaagccgctgtatgacgctctggtggtgcaatgccacaaagaagagtcaatcgcagacaacattttgaatgcggtcacacgttagcagcatgattgccacggatggcaacatattaacggcatgatattgacttattgaataaaattgggtaaatttgactcaacgatgggttaattcgctcgttgtggtagtgagatgaaaagaggcggcgcttactaccgattccgcctagttggtcacttcgacgtatcgtctggaactccaaccatcgcaggcagagaggtctgcaaaatgcaatcccgaaacagttcgcaggtaatagttagagcctgcataacggtttcgggattttttatatctgcacaacaggtaagagcattgagtcgataatcgtgaagagtcggcgagcctggttagccagtgctctttccgttgtgctgaattaagcgaataccggaagcagaaccggatcaccaaatgcgtacaggcgtcatcgccgcccagcaacagcacaacccaaactgagccgtagccactgtctgtcctgaattcattagtaatagttacgctgcggccttttacacatgaccttcgtgaaagcgggtggcaggaggtcgcgctaacaacctcctgccgttttgcccgtgcatatcggtcacgaacaaatctgattactaaacacagtagcctggatttgttctatcagtaatcgaccttattcctaattaaatagagcaaatccccttattgggggtaagacatgaagatgccagaaaaacatgacctgttggccgccattctcgcggcaaaggaacaaggcatcggggcaatccttgcgtttgcaatggcgtaccttcgcggcagatataatggcggtgcgtttacaaaaacagtaatcgacgcaacgatgtgcgccattatcgcctggttcattcgtgaccttctcgacttcgccggactaagtagcaatctcgcttatataacgagcgtgtttatcggctacatcggtactgactcgattggttcgcttatcaaacgcttcgctgctaaaaaagccggagtagaagatggtagaaatcaataatcaacgtaaggcgttcctcgatatgctggcgtggtcggagggaactgataacggacgtcagaaaaccagaaatcatggttatgacgtcattgtaggcggagagctatttactgattactccgatcaccctcgcaaacttgtcacgctaaacccaaaactcaaatcaacaggcgccggacgctaccagcttctttcccgttggtgggatgcctaccgcaagcagcttggcctgaaagacttctctccgaaaagtcaggacgctgtggcattgcagcagattaaggagcgtggcgctttacctatgattgatcgtggtgatatccgtcaggcaatcgaccgttgcagcaatatctgggcttcactgccgggcgctggttatggtcagttcgagcataaggctgacagcctgattgcaaaattcaaagaagcgggcggaacggtcagagagattgatgtatgagcagagtcaccgcgattatctccgctctggtcctgca

SEQ ID NO: 47 - DNA, 2594 bp, Artificial
  Molecule d'ADN double brin (1), variant (1.1), Exemple 12
gtaagagctgaggcggtgaccaatatctacaacatcagcctctcaagctgaggaagcggttagctccttcggtcctccgatcgttgtgtcattcatcaaggacgccgctatcgcaaatggtgctatccacgcagcggcaatcgaaacacctcagccggtgaccaatatctacaacatcagccttggtatccagcgtgatgagccagcgcagaacaaggtaaccgtcagtgccgataagttcaaagttaaacctggtgttgataccaacattgaaacgttgatcgaaaacgcgctgaaaaacgctgctgaatgtgcggcgctggatgtcacaaagcaaatggcagcagacaagaaagcgatggatgaactggcttcctatgtccgcacggccatcatgatggaatgtttccccggtggtgttatctggcagcagtgccgtcgatagtatgcaattgataattattatcatttgcgggtcctttccggcgatccgccttgttacggggcggcgacctcgcgggttttcgctatttatgaaaattttccggtttaaggcgtttccgttcttcttcgtcataacttaatgtttttatttaaaataccctctgaaaagaaaggaaacgacaggtgctgaaagcgagctttttggcctctgtcgtttcctttctctgtttttgtccgtggaatgaacaatggaagtcaacaaaaagcagctggctgacattttcggtgcgagtatccgtaccattcagaactggcaggaacagggaatgcccgttctgcgaggcggtggcaagggtaatgaggtgctttatgactctgccgccgtcataaaatggtatgccgaaagggatgctgaaattgagaacgaaaagctgcgccgggaggttgaagaactgcggcaggccaacgaggcagatccacaggacgggtgtggtcgccatgatcgcgtagtcgatagtggctccaagtagcgaagcgagcaggactgggcggcggccaaagcggtcggacagtgctccgagaacgggtgcgcatagaaattgcatcaacgcatatagcgctagcagcacgccatagtgactggcgatgctgtcggaatggacgatatcccgcaagaggcccggcagtaccggcataaccaagcctatgcctacagcatccagggtgacggtgccgaggatgacgatgagcgcattgttagatttcatacacggtgcctgactgcgttagcaatttaactgtgataaactaccgcattaaagcttgcatgcctgcatgcaggtcgacagtcagcagatgaacactgaccacaaggctgttttggataaggataatgcttatccagtggagtgctgggttcctgatccaagtaaaaatgaaaacactagatattttggaacctacacaggtggggaaaatgtgcctcctgttttgcacattactaacacagcaaccacagtgcttcttgatgagcagggtgttgggcccttgtgcaaagctgacagcttgtatgtttctgctgttgactctagaatatgatgaaagatagaaaattacgacgcttatcggaagtgaacgaatactttttatatgaggagggctgtttttacaaaatccggtagtaacttgctaaccaattcctaggcaggtcattggcaacagtggcatgcaccgagaaggacgtttgtaatgtccgctccggcacatagcagtcctagggacagtggcgtacagtcatagatggtcggtgggaggtggtacaaattctctcatgcaaaaaatatgtaaaatcggtagcaactggaaatcattcaacacccgcactatcggaagttcaccagccagccgcagcacgttcctgcatacgacgtgtctgcggctctaccatatctcctatgagcaacgtgttagcagagccaagccacaactctaattttaatacataatgaatgataataataatattaaaaatttcctgtgtaactaatttactatatggtttctgataagaatcattgcaaagatcaaacaacttgtattacattgacagttaagcagttaattttatcacctctaaaatatatcagcatctagcatgcaacctatcaaaatggagagttttatgactaaaaaaccatgggaaagaagacttaaagatttatcgcacttgctcaaatgctgcattgatacatattttgaccctgaattatttcgcttgaatttgaatcaattcctccaaaccgcaagaacagtaacatttattattcaaaaaaacaaaaaccagattataggatatgacatttggtataacaataatgttattgaaaaatggaaaaatgatccattaatggcttgggctaaaaattctcgcaatacgatagaaaaacaaggcgatttagaaatgtatagcgaggcaaaggctactcttatttcatcttacattgaagaaaatgacattgagtttattacaaatgaaagtatgttaaacattggtataaaaaagttagtcagacttgcacaaaagaaattaccttcatatttaactgaatcatctattattaaatcagaaagacgatgggtcgctaatacgc

SEQ ID NO: 48 - DNA, 2717 bp, Artificial
  Molecule d'ADN double brin (1), variant (1.2), Exemple 12
tctcaagctgaggaagcggttagctccttcggtcctccgatcgttgtgtcattcatcaaggacgccgctatcgcaaatggtgctatccacgcagcggcaatcgaaacacctcagccggtgaccaatatctacaacatcagccttggtatccagcgtgatgagccagcgcagaacaaggtaaccgtcagtgccgataagttcaaagttaaacctggtgttgataccaacattgaaacgttgatcgaaaacgcgctgaaaaacgctgctgaatgtgcggcgctggatgtcacaaagcaaatggcagcagacaagaaagcgatggatgaactggcttcctatgtccgcacggccatcatgatggaatgtttccccggtggtgttatctggcagcagtgccgtcgatagtatgcaattgataattattatcatttgcgggtcctttccggcgatccgccttgttacggggcggcgacctcgcgggttttcgctatttatgaaaattttccggtttaaggcgtttccgttcttcttcgtcataacttaatgtttttatttaaaataccctctgaaaagaaaggaaacgacaggtgctgaaagcgagctttttggcctctgtcgtttcctttctctgtttttgtccgtggaatgaacaatggaagtcaacaaaaagcagctggctgacattttcggtgcgagtatccgtaccattcagaactggcaggaacagggaatgcccgttctgcgaggcggtggcaagggtaatgaggtgctttatgactctgccgccgtcataaaatggtatgccgaaagggatgctgaaattgagaacgaaaagctgcgccgggaggttgaagaactgcggcaggccaacgaggcagatccacaggacgggtgtggtcgccatgatcgcgtagtcgatagtggctccaagtagcgaagcgagcaggactgggcggcggccaaagcggtcggacagtgctccgagaacgggtgcgcatagaaattgcatcaacgcatatagcgctagcagcacgccatagtgactggcgatgctgtcggaatggacgatatcccgcaagaggcccggcagtaccggcataaccaagcctatgcctacagcatccagggtgacggtgccgaggatgacgatgagcgcattgttagatttcatacacggtgcctgactgcgttagcaatttaactgtgataaactaccgcattaaagcttgcatgcctgcatgcaggtcgacagtcagcagatgaacactgaccacaaggctgttttggataaggataatgcttatccagtggagtgctgggttcctgatccaagtaaaaatgaaaacactagatattttggaacctacacaggtggggaaaatgtgcctcctgttttgcacattactaacacagcaaccacagtgcttcttgatgagcagggtgttgggcccttgtgcaaagctgacagcttgtatgtttctgctgttgactctagatccctctgaaaaaatcttccgagtttgctaggcactgatacataactcttttccaataattggggaagtcattcaaatctataataggtttcagatttgcttcaataaattctgactgtagctgctgaaacgttgcggttgaactatatttccttataacttttacgaaagagtttctttgagtaatcacttcactcaagtgcttccctgcctccaaacgatacctgttagcaatatttaatagcttgaaatgatgaagagctctgtgtttgtcttcctgcctccagttcgccgggcattcaacataaaaactgatagcacccggagttccggaaacgaaatttgcatatacccattgctcacgaaaaaaaatgtccttgtcgatatagggatgaatcgcttggtgtacctcatctactgcgaaaacttgacctttctctcccatattgcagtcgcggcacgatggaactaaattaataggcatcaccgaaaattcaggataatgtgcaataggaagaaaatgatctatattttttgtctgtcctatatcaccacaaaatggacatttttcacctgatgaaacaagcatgtcatcgtaatatgttctagcgggtttgtttttatctcggagattattttcataaagcttttctaatttaacctttgtcaggttaccaactactaaggttgtaggctcaagagggtgtgtcctgtcgtaggtaaataactgacctgtcgagcttaatattctatattgttgttctttctgcaaaaaagtggggaagtgagtaatgaaattatttctaacatttatctgcatcataccttccgagcatttattaagcatttcgctataagttctcgctggaagaggtagttttttcattgtactttaccttcatctctgttcattatcatcgcttttaaaacggttcgaccttctaatcctatctgaccattataattttttagaatggtttcataagaaagctctgaatcaacggactgcgataataagtggtggtatccagaatttgtcacttcaagtaaaaacacctcacgagttaaaacacctaagttctcaccgaatgtctcaatatccggacggataatatttattgcttctcttgaccgtaggactttccacatgcaggattttggaacctcttgcagtactactggggaatgagttgcaattattgctacaccattgcgtgcatc

SEQ ID NO: 49 - DNA, 2412 bp, Artificial
  Molecule d'ADN double brin (2), variant (2.1), Exemple 12
ttggtatccagcgtgatgagccagcgcagaacaaggtaaccgtcagtgccgataagttcaaagttaaacctggtgttgataccaacattgaaacgttgatcgaaaacgcgctgaaaaacgctgctgaatgtgcggcgctggatgtcacaaagcaaatggcagcagacaagaaagcgatggatgaactggcttcctatgtccgcacggccatcatgatggaatgtttccccggtggtgttatctggcagcagtgccgtcgatagtatgcaattgataattattatcatttgcgggtcctttccggcgatccgccttgttacggggcggcgacctcgcgggttttcgctatttatgaaaattttccggtttaaggcgtttccgttcttcttcgtcataacttaatgtttttatttaaaataccctctgaaaagaaaggaaacgacaggtgctgaaagcgagctttttggcctctgtcgtttcctttctctgtttttgtccgtggaatgaacaatggaagtcaacaaaaagcagctggctgacattttcggtgcgagtatccgtaccattcagaactggcaggaacagggaatgcccgttctgcgaggcggtggcaagggtaatgaggtgctttatgactctgccgccgtcataaaatggtatgccgaaagggatgctgaaattgagaacgaaaagctgcgccgggaggttgaagaactgcggcaggccaacgaggcagatccacaggacgggtgtggtcgccatgatcgcgtagtcgatagtggctccaagtagcgaagcgagcaggactgggcggcggccaaagcggtcggacagtgctccgagaacgggtgcgcatagaaattgcatcaacgcatatagcgctagcagcacgccatagtgactggcgatgctgtcggaatggacgatatcccgcaagaggcccggcagtaccggcataaccaagcctatgcctacagcatccagggtgacggtgccgaggatgacgatgagcgcattgttagatttcatacacggtgcctgactgcgttagcaatttaactgtgataaactaccgcattaaagcttgcatgcctgcatgcaggtcgacagtcagcagatgaacactgaccacaaggctgttttggataaggataatgcttatccagtggagtgctgggttcctgatccaagtaaaaatgaaaacactagatattttggaacctacacaggtggggaaaatgtgcctcctgttttgcacattactaacacagcaaccacagtgcttcttgatgagcagggtgttgggcccttgtgcaaagctgacagcttgtatgtttctgctgttgactctagaatatgatgaaagatagaaaattacgacgcttatcggaagtgaacgaatactttttatatgaggagggctgtttttacaaaatccggtagtaacttgctaaccaattcctaggcaggtcattggcaacagtggcatgcaccgagaaggacgtttgtaatgtccgctccggcacatagcagtcctagggacagtggcgtacagtcatagatggtcggtgggaggtggtacaaattctctcatgcaaaaaatatgtaaaatcggtagcaactggaaatcattcaacacccgcactatcggaagttcaccagccagccgcagcacgttcctgcatacgacgtgtctgcggctctaccatatctcctatgagcaacgtgttagcagagccaagccacaactctaattttaatacataatgaatgataataataatattaaaaatttcctgtgtaactaatttactatatggtttctgataagaatcattgcaaagatcaaacaacttgtattacattgacagttaagcagttaattttatcacctctaaaatatatcagcatctagcatgcaacctatcaaaatggagagttttatgactaaaaaaccatgggaaagaagacttaaagatttatcgcacttgctcaaatgctgcattgatacatattttgaccctgaattatttcgcttgaatttgaatcaattcctccaaaccgcaagaacagtaacatttattattcaaaaaaacaaaaaccagattataggatatgacatttggtataacaataatgttattgaaaaatggaaaaatgatccattaatggcttgggctaaaaattctcgcaatacgatagaaaaacaaggcgatttagaaatgtatagcgaggcaaaggctactcttatttcatcttacattgaagaaaatgacattgagtttattacaaatgaaagtatgttaaacattggtataaaaaagttagtcagacttgcacaaaagaaattaccttcatatttaactgaatcatctattattaaatcagaaagacgatgggtcgctaatacgc

SEQ ID NO: 50 - DNA, 2615 bp, Artificial
  Molecule d'ADN double brin (2), variant (2.2), Exemple 12
gtaagagctgaggcggtgaccaatatctacaacatcagccttggtatccagcgtgatgagccagcgcagaacaaggtaaccgtcagtgccgataagttcaaagttaaacctggtgttgataccaacattgaaacgttgatcgaaaacgcgctgaaaaacgctgctgaatgtgcggcgctggatgtcacaaagcaaatggcagcagacaagaaagcgatggatgaactggcttcctatgtccgcacggccatcatgatggaatgtttccccggtggtgttatctggcagcagtgccgtcgatagtatgcaattgataattattatcatttgcgggtcctttccggcgatccgccttgttacggggcggcgacctcgcgggttttcgctatttatgaaaattttccggtttaaggcgtttccgttcttcttcgtcataacttaatgtttttatttaaaataccctctgaaaagaaaggaaacgacaggtgctgaaagcgagctttttggcctctgtcgtttcctttctctgtttttgtccgtggaatgaacaatggaagtcaacaaaaagcagctggctgacattttcggtgcgagtatccgtaccattcagaactggcaggaacagggaatgcccgttctgcgaggcggtggcaagggtaatgaggtgctttatgactctgccgccgtcataaaatggtatgccgaaagggatgctgaaattgagaacgaaaagctgcgccgggaggttgaagaactgcggcaggccaacgaggcagatccacaggacgggtgtggtcgccatgatcgcgtagtcgatagtggctccaagtagcgaagcgagcaggactgggcggcggccaaagcggtcggacagtgctccgagaacgggtgcgcatagaaattgcatcaacgcatatagcgctagcagcacgccatagtgactggcgatgctgtcggaatggacgatatcccgcaagaggcccggcagtaccggcataaccaagcctatgcctacagcatccagggtgacggtgccgaggatgacgatgagcgcattgttagatttcatacacggtgcctgactgcgttagcaatttaactgtgataaactaccgcattaaagcttgcatgcctgcatgcaggtcgacagtcagcagatgaacactgaccacaaggctgttttggataaggataatgcttatccagtggagtgctgggttcctgatccaagtaaaaatgaaaacactagatattttggaacctacacaggtggggaaaatgtgcctcctgttttgcacattactaacacagcaaccacagtgcttcttgatgagcagggtgttgggcccttgtgcaaagctgacagcttgtatgtttctgctgttgactctagatccctctgaaaaaatcttccgagtttgctaggcactgatacataactcttttccaataattggggaagtcattcaaatctataataggtttcagatttgcttcaataaattctgactgtagctgctgaaacgttgcggttgaactatatttccttataacttttacgaaagagtttctttgagtaatcacttcactcaagtgcttccctgcctccaaacgatacctgttagcaatatttaatagcttgaaatgatgaagagctctgtgtttgtcttcctgcctccagttcgccgggcattcaacataaaaactgatagcacccggagttccggaaacgaaatttgcatatacccattgctcacgaaaaaaaatgtccttgtcgatatagggatgaatcgcttggtgtacctcatctactgcgaaaacttgacctttctctcccatattgcagtcgcggcacgatggaactaaattaataggcatcaccgaaaattcaggataatgtgcaataggaagaaaatgatctatattttttgtctgtcctatatcaccacaaaatggacatttttcacctgatgaaacaagcatgtcatcgtaatatgttctagcgggtttgtttttatctcggagattattttcataaagcttttctaatttaacctttgtcaggttaccaactactaaggttgtaggctcaagagggtgtgtcctgtcgtaggtaaataactgacctgtcgagcttaatattctatattgttgttctttctgcaaaaaagtggggaagtgagtaatgaaattatttctaacatttatctgcatcataccttccgagcatttattaagcatttcgctataagttctcgctggaagaggtagttttttcattgtactttaccttcatctctgttcattatcatcgcttttaaaacggttcgaccttctaatcctatctgaccattataattttttagaatggtttcataagaaagctctgaatcaacggactgcgataataagtggtggtatccagaatttgtcacttcaagtaaaaacacctcacgagttaaaacacctaagttctcaccgaatgtctcaatatccggacggataatatttattgcttctcttgaccgtaggactttccacatgcaggattttggaacctcttgcagtactactggggaatgagttgcaattattgctacaccattgcgtgcatc